European Patent Application EP 4 446 407 A1, published October 16, 2024. Title: ENGINEERED MICROORGANISM FOR TREATING HYPERPHENYLALANINEMIA AND USE THEREOF. Applicant: COMMBIO THERAPEUTICS CO., LTD. Application EP. The sequence listing filed with the application follows.

SEQUENCE LISTING (133 sequences)

SEQ ID NO: 1 - protein, 397 aa, synthetic construct
MFQKVDAYAGDPILTLMERFKEDPRSDKVNLSIGLYYNEDGIIPQLQAVAEAEARLNAQPHGASLYLPMEGLNSYRHAIAPLLFGADHPVLKQQRVATIQTLGGSGALKVGADFLKRYFPESGVWVSDPTWENHVAIFAGAGFEVSTYPWYDEATNGVRFNDLLATLKTLPARSIVLLHPCCHNPTGADLTNDQWDAVIEILKARELIPFLDIAYQGFGAGMEEDAYAIRAIASAGLPALVSNSFSKIFSLYGERVGGLSVMCEDAEAAGRVLGQLKATVRRNYSSPPNFGAQVVAAVLNDEALKASWLAEVEEMRTRILAMRQELVKVLSTEMPERNFDYLLNQRGMFSYTGLSAAQVDRLREEFGVYLIASGRMCVAGLNTANVQRVAKAFAAVM

SEQ ID NO: 2 - protein, 500 aa, synthetic construct
MTLPESKDFSYLFSDETNARKPSPLKTCIHLFQDPNIIFLGGGLPLKDYFPWDNLSVDSPKPPFPQGIGAPIDEQNCIKYTVNKDYADKSANPSNDIPLSRALQYGFSAGQPELLNFIRDHTKIIHDLKYKDWDVLATAGNTNAWESTLRVFCNRGDVILVEAHSFSSSLASAEAQGVITFPVPIDADGIIPEKLAKVMENWTPGAPKPKLLYTIPTGQNPTGTSIADHRKEAIYKIAQKYDFLIVEDEPYYFLQMNPYIKDLKEREKAQSSPKQDHDEFLKSLANTFLSLDTEGRVIRMDSFSKVLAPGTRLGWITGSSKILKPYLSLHEMTIQAPAGFTQVLVNATLSRWGQKGYLDWLLGLRHEYTLKRDCAIDALYKYLPQSDAFVINPPIAGMFFTVNIDASVHPEFKTKYNSDPYQLEQSLYHKVVERGVLVVPGSWFKSEGETEPPQPAESKEVSNPNIIFFRGTYAAVSPEKLTEGLKRLGDTLYEEFGISK

SEQ ID NO: 3 - protein, 379 aa, synthetic construct
MILVTLEQTLQDDKASVLDKMVEHEQILFCHDKATGLQAIIAVHDTTMGPALGGCRMAPYKTMDLALKDVLRLSKGMTYKCAAADVDFGGGKSVIIGDPLKDKTPEKFRAFGQFIESLNGRFYTGTDMGTTLEDFVHAMKETNYIVGKPVEYGGGGDSSIPTALGVFYGIKATNQNLFGDDKVEGRKYSIQGLGKVGYKVAEHIINEGGNVIVTDINEQAIADIQKLGGSAVRVVSSEEIYSQQADVFVPCAFGGVINDDTLKVLKVRGISGSANNQLAESRHGELLREKGILYAPDYIVNGGGLIQVADELYGTNPARVLAKTENIYTSLLEVFHQAEQDHMTTATAADRMCEKRIADAKNRNSFFTQSNRPKWNFHQ

SEQ ID NO: 4 - protein, 381 aa, synthetic construct
MAKQLEKSSKIGNEDVFQKIANHEQIVFCNDPVSGLQAIIAIHDTTLGPALGGTRMYPYKNVDEALEDVLRLSEGMTYKCAAADIDFGGGKAVIIGDPEKDKSPALFRAFGQFVESLNGRFYTGTDMGTTMDDFVHAQKETNFINGIPEQYGGSGDSSIPTAQGVIYALKATNQYLFGSDSLSGKTYAIQGLGKVGYKVAEQLLKAGADLFVTDIHENVLNSIKQKSEELGGSVTIVKSDDIYSVQADIFVPCAMGGIINDKTIPKLKVKAVVGSANNQLKDLRHANVLNEKGILYAPDYIVNAGGLIQVADELYGPNKERVLLKTKEIYRSLLEIFNQAALDCITTVEAANRKCQKTIEGQQTRNSFFSRGRRPKWNIKE

SEQ ID NO: 5 - protein, 380 aa, synthetic construct
MSLVEKTSIIKDFTLFEKMSEHEQVVFCNDPATGLRAIIAIHDTTLGPALGGCRMQPYNSVEEALEDALRLSKGMTYKCAASDVDFGGGKAVIIGDPQKDKSPELFRAFGQFVDSLGGRFYTGTDMGTNMEDFIHAMKETNCIVGVPEAYGGGGDSSIPTAMGVLYGIKATNKMLFGKDDLGGVTYAIQGLGKVGYKVAEGLLEEGAHLFVTDINEQTLEAIQEKAKTTSGSVTVVASDEIYSQEADVFVPCAFGGVVNDETMKQFKVKAIAGSANNQLLTEDHGRHLADKGILYAPDYIVNSGGLIQVADELYEVNKERVLAKTKHIYDAILEVYQQAELDQITTMEAANRMCEQRMAARGRRNSFFTSSVKPKWDIRN

SEQ ID NO: 6 - protein, 387 aa, synthetic construct
MASLSDKMKTFTKETEVRGMDMFDQIKNHEQVLFCNDEETGLKAIIAIHNTTLGPALGGCRMMPYASVDAALNDVLRLSRGMTYKCAAADVDFGGGKAVIIGDPTKDKHPELFRAFGQFVESLQGRFYTGTDMGTSPDDFVHALKETNCIVGVDEVYGGSGDSSIPTAMGVIYGLEATNETIWGSRDLHGKRYAIQGLGKVGFKVAERLLEEGADLIVTDISHHSVEKLQLKAKALGTAVKAVSGDEIYSVDADVFIPCAIGGILNDETIERLKVKAVAGSANNQLLEHRHGMSLHQRGILYAPDYIVNAGGLIQVADELYEPNKERVLQKTGAIYNSLLNIYTQSENEHITTVQAADRFCENRIQTRTKRNSFFTHTKRPKWSVRK

SEQ ID NO: 7 - protein, 635 aa, synthetic construct
MAPVTIEKFVNQEERHLVSNRSATIPFGEYIFKRLLSIDTKSVFGVPGDFNLSLLEYLYSPSVESAGLRWVGTCNELNAAYAADGYSRYSNKIGCLITTYGVGELSALNGIAGSFAENVKVLHIVGVAKSIDSRSSNFSDRNLHHLVPQLHDSNFKGPNHKVYHDMVKDRVACSVAYLEDIETACDQVDNVIRDIYKYSKPGYIFVPADFADMSVTCDNLVNVPRISQQDCIVYPSENQLSDIINKITSWIYSSKTPAILGDVLTDRYGVSNFLNKLICKTGIWNFSTVMGKSVIDESNPTYMGQYNGKEGLKQVYEHFELCDLVLHFGVDINEINNGHYTFTYKPNAKIIQFHPNYIRLVDTRQGNEQMFKGINFAPILKELYKRIDVSKLSLQYDSNVTQYTNETMRLEDPTNGQSSIITQVHLQKTMPKFLNPGDVVVCETGSFQFSVRDFAFPSQLKYISQGFFLSIGMALPAALGVGIAMQDHSNAHINGGNVKEDYKPRLILFEGDGAAQMTIQELSTILKCNIPLEVIIWNNNGYTIERAIMGPTRSYNDVMSWKWTKLFEAFGDFDGKYTNSTLIQCPSKLALKLEELKNSNKRSGIELLEVKLGELDFPEQLKCMVEAAALKRNKK

SEQ ID NO: 8 - protein, 549 aa, synthetic construct
MTNTVIKYVLDRLYDLGIKDIFGVAGDYAFPIEDTVCNNQQQRWIGNCNELNAAYAADGYARIKGMAALSTTFGVGELSAINAIAGAYAENLPIFHLVGMPASGVQKSKRLVHHTLGNGDFDVFYQIAQRLACAHTILTPENCVEEMERVIEAALKERRPVYIGIPSDYANSQVVAPLSVTAPQKPTSDKATLEKAVSAIIEKLTHSNNVCVLPGFLSARLGLTDKIQHFIDKTGLPYATMFMDKSILSESNTQYVGMYDGQLMTPEVREFVESSEYILGIGTLLTDFNTGSFTANIKSEQFISIMPDYVEIDSVIYSCVYMTDILSELTQRLPNKTYHKITAKGLGEAVTSDNNKITAQYLYPRLEQFFKPNDIIIAETGTSSMGLGFALLPEGAQFHNQTLWGSIGWATPAALGAALAAPEKRIILITGEGSHQLTVQEISQFVRFGLKPIILVLNNDGYLIERLLCDYPEAYYNDLAQWNYHQLPQAFGATDWYSEKVTTASGLDNALNKAALTNSASYIEIVTERYEASELAQNLKGSKSSLYSF

SEQ ID NO: 9 - protein, 349 aa, synthetic construct
MKIKAVGAYSAKQPLEPMDITRREPGPNDVKIEIAYCGVCHSDLHQVRSEWAGTVYPCVPGHEIVGRVVAVGDQVEKYAPGDLVGVGCIVDSCKHCEECEDGLENYCDHMTGTYNSPTPDEPGHTLGGYSQQIVVHERYVLRIRHPQEQLAAVAPLLCAGITTYSPLRHWQAGPGKKVGVVGIGGLGHMGIKLAHAMGAHVVAFTTSEAKREAAKALGADEVVNSRNADEMAAHLKSFDFILNTVAAPHNLDDFTTLLKRDGTMTLVGAPATPHKSPEVFNLIMKRRAIAGSMIGGIPETQEMLDFCAEHGIVADIEMIRADQINEAYERMLRGDVKYRFVIDNRTLTD

SEQ ID NO: 10 - protein, 477 aa, synthetic construct
MNTENIEQAIRKILSEELSNPQSSTATNTTVPGKNGIFKTVNEAIAATKAAQENYADQPISVRNKVIDAIREGFRPYIEDMAKRIHDETGMGTVSAKIAKLNNALYNTPGPEILQPEAETGDGGLVMYEYAPFGVIGAVGPSTNPSETVIANAIMMLAGGNTLFFGAHPGAKNITRWTIEKLNELVADATGLHNLVVSLETPSIESVQEVMQHPDVAMLSITGGPAVVHQALISGKKAVGAGAGNPPAMVDATANIALAAHNIVDSAAFDNNILCTAEKEVVVEAAVKDELIMRMQQEGAFLVTDSADIEKLAQMTIGPKGAPDRKFVGKDATYILDQAGISYTGTPTLIILEAAKDHPLVTTEMLMPILPVVCCPDFDSVLATATEVEGGLHHTASIHSENLPHINKAAHRLNTSIFVVNGPTYCGTGVATNGAHSGASALTIATPTGEGTATSKTYTRRRRLNSPEGFSLRTWEA

SEQ ID NO: 11 - protein, 1092 aa, synthetic construct
MLFDNKNRGALNSLNTPDIASLSISSMSDYHVFDFPGKDLQREEVIDLLDQQGFIPDDLIEQEVDWFYNSLGIDDLFFSRESPQLISNIIHSLYASKLDFFAKSKFNGIQPRLFSIKNKIITNDNHAIFMESNTGVSISDSQQKNFKFASDAVGNDTLEHGKDTIKKNRIEMDDSCPPYELDSEIDDLFLDNKSQKNCRLVSFWAPESELKLTFVYESVYPNDDPAGVDISSQDLLKGDIESISDKTMYKVSSNENKKLYGLLLKLVKEREGPVIKTTRSVENKDEIRLLVAYKRFTTKRYYSALNSLFHYYKLKPSKFYLESFNVKDDDIIIFSVYLNENQQLEDVLLHDVEAALKQVEREASLLYAIPNNSFHEVYQRRQFSPKEAIYAHIGAIFINHFVNRLGSDYQNLLSQITIKRNDTTLLEIVENLKRKLRNETLTQQTIINIMSKHYTIISKLYKNFAQIHYYHNSTKDMEKTLSFQRLEKVEPFKNDQEFEAYLNKFIPNDSPDLLILKTLNIFNKSILKTNFFITRKVAISFRLDPSLVMTKFEYPETPYGIFFVVGNTFKGFHIRFRDIARGGIRIVCSRNQDIYDLNSKNVIDENYQLASTQQRKNKDIPEGGSKGVILLNPGLVEHDQTFVAFSQYVDAMIDILINDPLKENYVNLLPKEEILFFGPDEGTAGFVDWATNHARVRNCPWWKSFLTGKSPSLGGIPHDEYGMTSLGVRAYVNKIYETLNLTNSTVYKFQTGGPDGDLGSNEILLSSPNECYLAILDGSGVLCDPKGLDKDELCRLAHERKMISDFDTSKLSNNGFFVSVDAMDIMLPNGTIVANGTTFRNTFHTQIFKFVDHVDIFVPCGGRPNSITLNNLHYFVDEKTGKCKIPYIVEGANLFITQPAKNALEEHGCILFKDASANKGGVTSSSMEVLASLALNDNDFVHKFIGDVSGERSALYKSYVVEVQSRIQKNAELEFGQLWNLNQLNGTHISEISNQLSFTINKLNDDLVASQELWLNDLKLRNYLLLDKIIPKILIDVAGPQSVLENIPESYLKVLLSSYLSSTFVYQNGIDVNIGKFLEFIGGLKREAEASA

SEQ ID NO: 12 - protein, 421 aa, synthetic construct
MSGKDVNVFEMAQSQVKNACDKLGMEPAVYELLKEPMRVIEVSIPVKMDDGSIKTFKGFRSQHNDAVGPTKGGIRFHQNVSRDEVKALSIWMTFKCSVTGIPYGGGKGGIIVDPSTLSQGELERLSRGYIDGIYKLIGEKVDVPAPDVNTNGQIMSWMVDEYNKLTGQSSIGVITGKPVEFGGSLGRTAATGFGVAVTAREAAAKLGIDMKKAKIAVQGIGNVGSYTVLNCEKLGGTVVAMAEWCKSEGSYAIYNENGLDGQAMLDYMKEHGNLLNFPGAKRISLEEFWASDVDIVIPAALENSITKEVAESIKAKLVCEAANGPTTPEADEVFAERGIVLTPDILTNAGGVTVSYFEWVQNLYGYYWSEEEVEQKEEIAMVKAFESIWKIKEEYNVTMREAAYMHSIKKVAEAMKLRGWY

SEQ ID NO: 13 - protein, 460 aa, synthetic construct
MKNASTVSEDTASNQEPTLHRGLHNRHIQLIALGGAIGTGLFLGIGPAIQMAGPAVLLGYGVAGIIAFLIMRQLGEMVVEEPVSGSFAHFAYKYWGPFAGFLSGWNYWVMFVLVGMAELTAAGIYMQYWFPDVPTWIWAAAFFIIINAVNLVNVRLYGETEFWFALIKVLAIIGMIGFGLWLLFSGHGGEKASINNLWRYGGFFATGWNGLILSLAVIMFSFGGLELIGITAAEARDPEKSIPKAVNQVVYRILLFYIGSLVVLLALYPWVEVKSNSSPFVMIFHNLDSNVVASALNFVILVASLSVYNSGVYSNSRMLFGLSVQGNAPKFLTRVSRRGVPINSLMLSGAITSLVVLINYLLPQKAFGLLMALVVATLLLNWIMICLAHLRFRAAMRRQGRETQFKALLYPFGNYLCIAFLGMILLLMCTMDDMRLSAILLPVWIVFLFVAFKTLRRKVN

SEQ ID NO: 14 - protein, 460 aa, synthetic construct
MKNASTVSEDTASNQEPTLHRGLHNRHIQLIALGGAIGTGLFLGIGPAIQMAGPAVLLGYGVAGIIAFLIMRQLGEMVVEEPVSGSFAHFAYKYWGPFAGFLSGWNYWVMYVLVGMAELTAAGIYMQYWFPDVPTWIWAAAFFIIINAVNLVNVRLYGETEFWFALIKVLAIIGMIGFGLWLLFSGHGGEKASINNLWRYGGFFATGWNGLILSLAVIMFSFGGLELIGITAAEARDPEKSIPKAVNQVVYRILLFYIGSLVVLLALYPWVEVKSNSSPFVMIFHNLDSNVVASALNFVILVASLSVYNSGVYSNSRMLFGLSVQGNAPKFLTRVSRRGVPINSLMLSGAITSLVVLINYLLPQKAFGLLMALVVATLLLNWIMICLAHLRFRAAMRRQGRETQFKALLYPFGNYLCIAFLGMILLLMCTMDDMRLSAILLPVWIVFLFVAFKTLRRKVN

SEQ ID NO: 15 - DNA, 1194 bp, synthetic construct
  source 1..1194: mol_type = other DNA
gtgtttcaaaaagttgacgcctacgctggcgacccgattcttacgcttatggagcgttttaaagaagaccctcgcagcgacaaagtgaatttaagtatcggtctgtactacaacgaagacggaattattccacaactgcaagccgtggcggaggcggaagcgcgcctgaatgcgcagcctcatggcgcttcgctttatttaccgatggaagggcttaacagctatcgccatgccattgcgccgctgctgtttggtgcggaccatccggtactgaaacaacagcgcgtagcaaccattcaaacccttggcggctccggggcattgaaagtgggcgcggatttcctgaaacgctacttcccggaatcaggcgtctgggtcagcgatcctacctgggaaaaccacgtagcaatattcgccggggctggattcgaagtgagtacttacccctggtatgacgaagcgactaacggcgtgcgctttaatgacctgttggcgacgctgaaaacattacctgcccgcagtattgtgttgctgcatccatgttgccacaacccaacgggtgccgatctcactaatgatcagtgggatgcggtgattgaaattctcaaagcccgcgagcttattccattcctcgatattgcctatcaaggatttggtgccggtatggaagaggatgcctacgctattcgcgccattgccagcgctggattacccgctctggtgagcaattcgttctcgaaaattttctccctttacggcgagcgcgtcggcggactttctgttatgtgtgaagatgccgaagccgctggccgcgtactggggcaattgaaagcaacagttcgccgcaactactccagcccgccgaattttggtgcgcaggtggtggctgcagtgctgaatgacgaggcattgaaagccagctggctggcggaagtagaagagatgcgtactcgcattctggcaatgcgtcaggaattggtgaaggtattaagcacagagatgccagaacgcaatttcgattatctgcttaatcagcgcggcatgttcagttataccggtttaagtgccgctcaggttgaccgactacgtgaagaatttggtgtctatctcatcgccagcggtcgcatgtgtgtcgccgggttaaatacggcaaatgtacaacgtgtggcaaaggcgtttgctgcggtgatgtaa

SEQ ID NO: 16 - DNA, 1164 bp, synthetic construct
  source 1..1164: mol_type = other DNA
atggcaagcctatccgataaaatgaaaacgtttacaaaagagacggaggtcagggggatggacatgttcgaccagatcaagaatcatgaacaggtcctgttctgcaacgatgaagagaccggtttgaaagcgatcatcgccatacataataccactctcggacctgcactcggcgggtgccggatgatgccgtatgcctcagtggatgcggcattgaacgacgtactcagattgtcgagggggatgacatacaaatgcgcggcggcagacgtggactttggcggggggaaggcggtcatcatcggtgacccgaccaaagataaacatcccgagctgttcagggcattcgggcaattcgtcgaatcccttcagggaaggttctacacagggacggatatgggcacgtcgccggatgattttgtccacgccctgaaggaaaccaactgcatcgtcggtgtcgatgaagtatatggcggaagtggagattcttcgattccgacagccatgggtgtcatctatggacttgaagccacgaacgaaaccatctggggatcaagggatcttcatgggaagcgctatgcgattcaggggcttgggaaagtcggattcaaagtagcggaacgtctccttgaggaaggggccgatctaattgtgaccgatatcagtcatcactcagttgaaaaactgcagctgaaagcaaaagccctcggaacggcagtgaaggccgtcagcggagacgaaatctactcagtggatgccgatgtgttcatcccttgtgccataggagggatcctgaacgacgagacaatcgaaaggttaaaggtaaaagccgtcgccggttctgccaataatcagctcctcgagcaccgacacgggatgtcccttcatcaaagggggatcctgtatgcccctgattacatcgttaatgcaggcggcctaatccaggtagccgatgaactctatgaacctaacaaagaacgcgtcctccagaaaacaggagccatctataacagcctcctcaacatctacacccaatcagaaaacgaacacatcaccaccgtccaagcagcagaccgcttctgcgaaaaccgcatccaaaccagaaccaaacgaaacagcttcttcacccacaccaaacgcccaaaatggagtgtaaggaagtaa

SEQ ID NO: 17 - DNA, 1164 bp, synthetic construct
  source 1..1164: mol_type = other DNA
atggcgagcctgagcgataagatgaagacctttaccaaggagaccgaagtgcgtggcatggatatgtttgaccagatcaagaatcacgaacaggttctgttttgcaacgacgaggaaaccggcctgaaggcgatcattgcgattcacaacaccaccctgggtccggcgctgggtggctgccgtatgatgccgtatgcgagcgtggatgcggcgctgaacgatgttctgcgtctgagccgtggcatgacctataagtgcgcggcggcggatgtggattttggtggcggtaaagcggttatcattggtgacccgaccaaggataaacacccggagctgttccgtgcgtttggccagttcgtggaaagcctgcaaggtcgtttttacaccggtaccgacatgggtaccagcccggacgatttcgtgcacgcgctgaaggaaaccaactgcatcgtgggcgttgacgaagtttacggcggtagcggtgatagcagcatcccgaccgcgatgggcgtgatttatggtctggaggcgaccaacgaaaccatttggggcagccgtgatctgcacggtaaacgttacgcgatccagggcctgggcaaagtgggctttaaagttgcggagcgtctgctggaggaaggtgctgacctgatcgtgaccgatattagccaccacagcgttgaaaagctgcaactgaaggcgaaagcgctgggcaccgcggtgaaagcggttagcggtgacgagatttatagcgtggacgcggatgttttcatcccgtgcgcgatcggcggtattctgaacgatgaaaccatcgaacgtctgaaggtgaaagcggtggcgggtagcgcgaacaaccagctgctggagcaccgtcacggcatgagcctgcaccaacgtggtatcctgtacgcgccggactatattgtgaacgcgggcggtctgatccaggttgcggatgagctgtatgaaccgaacaaggaacgtgttctgcaaaaaaccggtgcgatttacaacagcctgctgaacatctatacccagagcgagaacgaacacattaccaccgtgcaagcggcggatcgtttttgcgagaaccgtatccaaacccgtaccaagcgtaacagctttttcacccataccaaacgtccgaagtggagcgtgcgtaaataa

SEQ ID NO: 18 - DNA, 1908 bp, synthetic construct
  source 1..1908: mol_type = other DNA
atggcacctgttacaattgaaaagttcgtaaatcaagaagaacgacaccttgtttccaaccgatcagcaacaattccgtttggtgaatacatatttaaaagattgttgtccatcgatacgaaatcagttttcggtgttcctggtgacttcaacttatctctattagaatatctctattcacctagtgttgaatcagctggcctaagatgggtcggcacgtgtaatgaactgaacgccgcttatgcggccgacggatattcccgttactctaataagattggctgtttaataaccacgtatggcgttggtgaattaagcgccttgaacggtatagccggttcgttcgctgaaaatgtcaaagttttgcacattgttggtgtggccaagtccatagattcgcgttcaagtaactttagtgatcggaacctacatcatttggtcccacagctacatgattcaaattttaaagggccaaatcataaagtatatcatgatatggtaaaagatagagtcgcttgctcggtagcctacttggaggatattgaaactgcatgtgaccaagtcgataatgttatccgcgatatttacaagtattctaaacctggttatatttttgttcctgcagattttgcggatatgtctgttacatgtgataatttggttaatgttccacgtatatctcaacaagattgtatagtatacccttctgaaaaccaattgtctgacataatcaacaagattactagttggatatattccagtaaaacacctgcgatccttggagacgtactgactgataggtatggtgtgagtaactttttgaacaagcttatctgcaaaactgggatttggaatttttccactgttatgggaaaatctgtaattgatgagtcaaacccaacttatatgggtcaatataatggtaaagaaggtttaaaacaagtctatgaacattttgaactgtgcgacttggtcttgcattttggagtcgacatcaatgaaattaataatgggcattatacttttacttataaaccaaatgctaaaatcattcaatttcatccgaattatattcgccttgtggacactaggcagggcaatgagcaaatgttcaaaggaatcaattttgcccctattttaaaagaactatacaagcgcattgacgtttctaaactttctttgcaatatgattcaaatgtaactcaatatacgaacgaaacaatgcggttagaagatcctaccaatggacaatcaagcattattacacaagttcacttacaaaagacgatgcctaaatttttgaaccctggtgatgttgtcgtttgtgaaacaggctcttttcaattctctgttcgtgatttcgcgtttccttcgcaattaaaatatatatcgcaaggatttttcctttccattggcatggcccttcctgccgccctaggtgttggaattgccatgcaagaccactcaaacgctcacatcaatggtggcaacgtaaaagaggactataagccaagattaattttgtttgaaggtgacggtgcagcacagatgacaatccaagaactgagcaccattctgaagtgcaatattccactagaagttatcatttggaacaataacggctacactattgaaagagccatcatgggccctaccaggtcgtataacgacgttatgtcttggaaatggaccaaactatttgaagcattcggagacttcgacggaaagtatactaatagcactctcattcaatgtccctctaaattagcactgaaattggaggagcttaagaattcaaacaaaagaagcgggatagaacttttagaagtcaaattaggcgaattggatttccccgaacagctaaagtgcatggttgaagcagcggcacttaaaagaaataaaaaatag

SEQ ID NO: 19 - DNA, 1050 bp, synthetic construct
  source 1..1050: mol_type = other DNA
atgaagatcaaagctgttggtgcatattccgctaaacaaccacttgaaccgatggatatcacccggcgtgaaccgggaccgaatgatgtcaaaatcgaaatcgcttactgtggcgtttgccattccgatctccaccaggtccgttccgagtgggcggggacggtttacccctgcgtgccgggtcatgaaattgtggggcgtgtggtagccgttggtgatcaggtagaaaaatatgcgccgggcgatctggtcggtgtcggctgcattgtcgacagttgtaaacattgcgaagagtgtgaagacgggttggaaaactactgtgatcacatgaccggcacctataactcgccgacgccggacgaaccgggccatactctgggcggctactcacaacagatcgtcgttcatgagcgatatgttctgcgtattcgtcacccgcaagagcagctggcggcggtggctcctttgttgtgtgcagggatcaccacgtattcgccgctacgtcactggcaggccgggccgggtaaaaaagtgggcgtggtcggcatcggcggtctgggacatatggggattaagctggcccacgcgatgggggcacatgtggtggcatttaccacttctgaggcaaaacgcgaagcggcaaaagccctgggggccgatgaagttgttaactcacgcaatgccgatgagatggcggctcatctgaagagtttcgatttcattttgaatacagtagctgcgccacataatctcgacgattttaccaccttgctgaagcgtgatggcaccatgacgctggttggtgcgcctgcgacaccgcataaatcgccggaagttttcaacctgatcatgaaacgccgtgcgatagccggttctatgattggcggcattccagaaactcaggagatgctcgatttttgcgccgaacatggcatcgtggctgatatagagatgattcgggccgatcaaattaatgaagcctatgagcgaatgctgcgcggtgatgtgaaatatcgttttgttatcgataatcgcacactaacagactga

SEQ ID NO: 20 - DNA, 1266 bp, synthetic construct
  source 1..1266: mol_type = other DNA
atgtcaggaaaagatgtaaatgtcttcgagatggcgcaatctcaagtaaaaaatgcatgtgataaattaggtatggaaccagcagtttatgaattattaaaagaacctatgagagttatagaggtttcaattccagtaaaaatggatgatggttctataaaaacttttaaaggatttagatcacaacataatgatgcagtagggccaacaaaaggtggaataagattccatcaaaatgtttcaagagacgaagtaaaagctttatctatatggatgactttcaagtgttctgtaacaggtataccatatggtggaggtaaaggtggaataatagtagatccatcaactttatctcaaggtgaattagaaagattaagtagaggatacatagatggaatatataaattaataggtgagaaagttgacgttcctgcaccagacgtaaatactaatggtcaaataatgtcttggatggttgatgagtacaataaattaactggacaaagttctataggtgttataactggtaagccagttgaatttggtggttctttaggaagaacagctgctactggatttggtgttgctgttacagcaagagaagctgctgctaaattaggaatagatatgaaaaaagctaaaatagctgttcaaggtataggaaacgttggttcttatacagttcttaactgtgaaaaacttggtggtactgttgtagctatggctgaatggtgtaaatcagaaggttcttatgctatatacaatgaaaatggtttagatggtcaagctatgttagattatatgaaagaacatggtaacttattaaacttcccaggagctaagagaatatctttagaagagttctgggcttcagatgttgatatagtaataccagctgcattagaaaactctataactaaagaagttgctgaatctataaaagctaaattagtttgtgaggctgctaatggaccaactactccagaggctgatgaagtatttgctgaaagaggaatagttcttactccagatatattaactaatgctggtggagttacagtttcttactttgagtgggtacaaaacttatatggatactactggtcagaagaagaagtagagcaaaaagaagaaatagctatggttaaagcatttgaatctatttggaaaatcaaagaagagtacaatgttacaatgagagaagctgcttacatgcattcaattaagaaagttgctgaagctatgaaattaagaggatggtactaa

SEQ ID NO: 21 - DNA, 1383 bp, synthetic construct
  source 1..1383: mol_type = other DNA
atgaaaaacgcgtcaaccgtatcggaagatactgcgtcgaatcaagagccgacgcttcatcgcggattacataaccgtcatattcaactgattgcgctgggtggcgcaattggtactggtctgtttcttggcattggcccggcgattcagatggcgggtccggctgtattgctgggctacggcgtcgccgggatcatcgctttcctgattatgcgccagctcggcgagatggtggtcgaagagccggtatccggttcatttgcccactttgcctataaatactggggaccgtttgcgggcttcctctctggctggaactactgggtaatgttcgtgctggtgggaatggcagagctgaccgctgcgggcatctatatgcagtactggttcccggatgttccaacgtggatttgggctgccgccttctttattatcatcaacgccgttaacctggtgaacgtgcgcttatatggcgaaaccgagttctggtttgcgctgattaaagtgctggcgatcatcggtatgatcggctttggcctgtggctgctgttttctgggcacggcggtgagaaagccagtatcaataacctctggcgctacggcggtttctttgccaccggctggaatggattgattttgtcgctggcggtaattatgttctccttcggcggtctggagctgattgggattactgcggctgaagcgcgcgatccggaaaaaagcatccctaaagcagtgaatcaggtggtgtatcgcatcctgctgttttatatcggttcactggtggttttactggcgctctacccgtgggtggaagtgaaatccaacagtagcccgtttgtgatgattttccataatctcgacagcaacgtggtagcttctgcgctgaacttcgtcattctggtggcatcgctgtcggtgtataacagcggggtttactctaacagccgcatgctgtttggcctttctgtgcagggtaatgcgccaaagtttttgactcgcgtcagccgtcgcggcgtgccgattaactcgctgatgctttccggagcgatcacttcgctggtggtgttaatcaactatctgctgccgcaaaaagcgtttggtctgctgatggcgctggtggtagcaacgctgctgttgaactggattatgatctgcctggcgcatctgcgttttcgtgcagcgatgcgtcgtcaggggcgtgaaacacagtttaaggcgctgctctatccgttcggcaactatctttgcatcgccttcctcggcatgattttgctgctgatgtgcacgatggatgatatgcgcttgtcagcgattctgctgccggtgtggattgtgttcctgtttgtggcgtttaaaacattgcgtaggaaagtgaattaa

SEQ ID NO: 22 - DNA, 624 bp, synthetic construct
  source 1..624: mol_type = other DNA
gacgtcccatggctcgagcatgcgagagtagggaactgccaggcatcaaataaaatgaaaggctcagtcgaaagactgggcctttcgttttatctgttgtttgtcggtgaacgctctcctgagtaggacaaatccgccgggagcggatttgaacgttgcgaagcaacggcccggagggtggcgggcaggacgcccgccataaactgccaggcatcaaattaagcagaaggccatcctgacggatggcctttttgcgtggccagtgccaagcttgcatgcagattgcagcattacacgtcttgagcgattgtgtaggctggagctgcttcgaagttcctatactttctagagaataggaacttcggaataggaactaaggaggatattcatatggaccatggctaattcccaggtaccagttgttcttattggtggtgttgctttatggttgcatcgtagtaaatggttgtaacaaaagcaatttttccggctgtctgtatacaaaaacgccgtaaagtttgagcgaagtcaataaactctctacccattcagggcaatatctctcttggatccaaagtgaactctagaaataattttgtttaactttaagaaggagatatacat

SEQ ID NO: 23 - DNA, 65 bp, synthetic construct
  source 1..65: mol_type = other DNA
aaaaacgccgcaaagtttgagcgaagtcaataaactctctacccattcagggcaatatctctctt

SEQ ID NO: 24 - DNA, 99 bp, synthetic construct
  source 1..99: mol_type = other DNA
tgaataaatagtgcccgtaatatcagggaatgaccccacataaaatgtggcataaaagatgcatactgtagtcgagagcgcgtatgcgtgatttgatta

SEQ ID NO: 25 - DNA, 33 bp, synthetic construct
  source 1..33: mol_type = other DNA
ctgcaggaattcaaaaaaagcaccgactcggtg

SEQ ID NO: 26 - DNA, 52 bp, synthetic construct
  source 1..52: mol_type = other DNA
actagtcgtatatcgaagatgtgacggttttagagctagaaatagcaagtta

SEQ ID NO: 27 - DNA, 20 bp, synthetic construct
  source 1..20: mol_type = other DNA
cctgattctgtggataaccg

SEQ ID NO: 28 - DNA, 45 bp, synthetic construct
  source 1..45: mol_type = other DNA
gagataaacccatcaggagaggacgtcccatggctcgagcatgcg

SEQ ID NO: 29 - DNA, 50 bp, synthetic construct
  source 1..50: mol_type = other DNA
tgggcaaaaacacgcgcttatgcttgcaggaaacacagaaaaaagcccgc

SEQ ID NO: 30 - DNA, 47 bp, synthetic construct
  source 1..47: mol_type = other DNA
ttcgcggccgcatctagagtaagcgcaacgtagaacaggaattattc

SEQ ID NO: 31 - DNA, 46 bp, synthetic construct
  source 1..46: mol_type = other DNA
atgctcgagccatgggacgtcctctcctgatgggtttatctcttac

SEQ ID NO: 32 - DNA, 48 bp, synthetic construct
  source 1..48: mol_type = other DNA
ggcttttttctgtgtttcctgcaagcataagcgcgtgtttttgcccag

SEQ ID NO: 33 - DNA, 37 bp, synthetic construct
  source 1..37: mol_type = other DNA
gtgactctagtattcatcgacgcgatgagagtaaaag

SEQ ID NO: 34 - DNA, 23 bp, synthetic construct
  source 1..23: mol_type = other DNA
gatatcatgatactgcggcgggg

SEQ ID NO: 35 - DNA, 24 bp, synthetic construct
  source 1..24: mol_type = other DNA
gctctggcgagtaagaggagatcc

SEQ ID NO: 36 - DNA, 33 bp, synthetic construct; identical to SEQ ID NO: 25
  source 1..33: mol_type = other DNA

SEQ ID NO: 37 - DNA, 56 bp, synthetic construct
  source 1..56: mol_type = other DNA
taatactagtcgatccgtatccaagtgcgggttttagagctagaaatagcaagtta

SEQ ID NO: 38 - DNA, 50 bp, synthetic construct
  source 1..50: mol_type = other DNA
tttgtttaactttaagaaggagatatacatatggcacctgttacaattga

SEQ ID NO: 39 - DNA, 63 bp, synthetic construct
  source 1..63: mol_type = other DNA
aacatcactggagaaagtcttatgaaactcgcaggaaacacagaaaaaagcccgcacctgaca

SEQ ID NO: 40 - DNA, 28 bp, synthetic construct
  source 1..28: mol_type = other DNA
tttcagcatttcgctaatggtgttatcg

SEQ ID NO: 41 - DNA, 26 bp, synthetic construct
  source 1..26: mol_type = other DNA
acgctgcaaaacttaagcaatctgga

SEQ ID NO: 42 - DNA, 27 bp, synthetic construct
  source 1..27: mol_type = other DNA
gagtttcataagactttctccagtgat

SEQ ID NO: 43 - DNA, 45 bp, synthetic construct
  source 1..45: mol_type = other DNA
gagccagtgtgactctagtaatcaagttctaccgtgccgacgttc

SEQ ID NO: 44 - DNA, 20 bp, synthetic construct
  source 1..20: mol_type = other DNA
ttaaaccagttcgttcgggc

SEQ ID NO: 45 - DNA, 20 bp, synthetic construct
  source 1..20: mol_type = other DNA
cgctattttcctgccagtcc

SEQ ID NO: 46 - DNA, 33 bp, synthetic construct; identical to SEQ ID NO: 25
  source 1..33: mol_type = other DNA

SEQ ID NO: 47 - DNA, 56 bp, synthetic construct
  source 1..56: mol_type = other DNA
taatactagtattgtggaaagaccacaccggttttagagctagaaatagcaagtta

SEQ ID NO: 48 - DNA, 60 bp, synthetic construct
  source 1..60: mol_type = other DNA
gcgttacatacctgatgcggctacgacgtcccatggctcgagcatgcgagagtagggaac

SEQ ID NO: 49 - DNA, 39 bp, synthetic construct
  source 1..39: mol_type = other DNA
gtaccttatcaagcacttgcctccgcttctctttttaac

SEQ ID NO: 50 - DNA, 27 bp, synthetic construct
  source 1..27: mol_type = other DNA
gtaatgcctgatagagcagccggtgag

SEQ ID NO: 51 - DNA, 33 bp, synthetic construct
  source 1..33: mol_type = other DNA
gacgtcgtagccgcatcaggtatgtaacgcctg

SEQ ID NO: 52 - DNA, 47 bp, synthetic construct
  source 1..47: mol_type = other DNA
gcttttttctgtgtttcctgccgtttcactccatccaaaaaaacggg

SEQ ID NO: 53 - DNA, 32 bp, synthetic construct
  source 1..32: mol_type = other DNA
gtgaaacggcaggaaacacagaaaaaagcccg

SEQ ID NO: 54 - DNA, 25 bp, synthetic construct
  source 1..25: mol_type = other DNA
gcagggaatggtgccgtagaaatag

SEQ ID NO: 55 - DNA, 22 bp, synthetic construct
  source 1..22: mol_type = other DNA
gtgagcctccggatgacgaccg

SEQ ID NO: 56 - DNA, 33 bp, synthetic construct; identical to SEQ ID NO: 25
  source 1..33: mol_type = other DNA

SEQ ID NO: 57 - DNA, 56 bp, synthetic construct
  source 1..56: mol_type = other DNA
taatactagtcgaagccgccctgtaaacgggttttagagctagaaatagcaagtta

SEQ ID NO: 58 - DNA, 46 bp, synthetic construct
  source 1..46: mol_type = other DNA
gcttattacccagctcgatgcaagacgtcccatggctcgagcatgc

SEQ ID NO: 59 - DNA, 34 bp, synthetic construct
  source 1..34: mol_type = other DNA
catctggtcgcaggaaacacagaaaaaagcccgc

SEQ ID NO: 60 - DNA, 40 bp, synthetic construct
  source 1..40: mol_type = other DNA
gccgcatctagagttatacatgtctgacaatggcagatcc

SEQ ID NO: 61 - DNA, 30 bp, synthetic construct
  source 1..30: mol_type = other DNA
gacgtcttgcatcgagctgggtaataagcg

SEQ ID NO: 62 - DNA, 45 bp, synthetic construct
  source 1..45: mol_type = other DNA
gcttttttctgtgtttcctgcgaccagatgatcacactcgggtga

SEQ ID NO: 63 - DNA, 40 bp, synthetic construct
  source 1..40: mol_type = other DNA
gtgtgactctagtacactacgcctgaacgttgaaaatccg

SEQ ID NO: 64 - DNA, 25 bp, synthetic construct
  source 1..25: mol_type = other DNA
gtgtgggccataattcaattcgcgc

SEQ ID NO: 65 - DNA, 24 bp, synthetic construct
  source 1..24: mol_type = other DNA
gaagttcagatgtacggcgagctg

SEQ ID NO: 66 - DNA, 33 bp, synthetic construct; identical to SEQ ID NO: 25
  source 1..33: mol_type = other DNA

SEQ ID NO: 67 - DNA, 55 bp, synthetic construct
  source 1..55: mol_type = other DNA
taatactagtgccggaagacactatgaagcgttttagagctagaaatagcaagtt

SEQ ID NO: 68 - DNA, 46 bp, synthetic construct
  source 1..46: mol_type = other DNA
cgcttattccagggcgaccagatgacgtcccatggctcgagcatgc

SEQ ID NO: 69 - DNA, 40 bp, synthetic construct
  source 1..40: mol_type = other DNA
ttaattcactttcctacgcaatgttttaaacgccacaaac

SEQ ID NO: 70 - DNA, 40 bp, synthetic construct
  source 1..40: mol_type = other DNA
tctggaattcgcggccgcatttgtttatggatgcgctggg

SEQ ID NO: 71 - DNA, 31 bp, synthetic construct
  source 1..31: mol_type = other DNA
atctggtcgccctggaataagcgttgtgaag

SEQ ID NO: 72 - DNA, 45 bp, synthetic construct
  source 1..45: mol_type = other DNA
attgcgtaggaaagtgaattaattgcatattcttgcgcgagcgcg

SEQ ID NO: 73 - DNA, 40 bp, synthetic construct
  source 1..40: mol_type = other DNA
gctttttttgaattcctgcaactcaaattcatcccagccg

SEQ ID NO: 74 - DNA, 20 bp, synthetic construct
  source 1..20: mol_type = other DNA
cagtcgaaatgttcgtctgc

SEQ ID NO: 75 - DNA, 20 bp, synthetic construct
  source 1..20: mol_type = other DNA
gcacaggattcaatggcgat

SEQ ID NO: 76 - DNA, 26 bp, synthetic construct
  source 1..26: mol_type = other DNA
acgctgcaaaacttaagcaatctgga

SEQ ID NO: 77 - DNA, 50 bp, synthetic construct
  source 1..50: mol_type = other DNA
tttttccagattgcttaagttttgcagcgtgacgtcccatggctcgagca

SEQ ID NO: 78 - DNA, 39 bp, synthetic construct
  source 1..39: mol_type = other DNA
gaaactcttaattcactttcctacgcaatgttttaaacg

SEQ ID NO: 79 - DNA, 51 bp, synthetic construct
  source 1..51: mol_type = other DNA
acattgcgtaggaaagtgaattaagagtttcataagactttctccagtgat

SEQ ID NO: 80 - DNA, 46 bp, synthetic construct; identical to SEQ ID NO: 31
  source 1..46: mol_type = other DNA

SEQ ID NO: 81 - DNA, 52 bp, synthetic construct
  source 1..52: mol_type = other DNA
gtaagagataaacccatcaggagaggacgtcccatggctcgagcatgcgaga

SEQ ID NO: 82 - DNA, 38 bp, synthetic construct
  source 1..38: mol_type = other DNA
cgcgcttatgcttgcaggaaacacagaaaaaagcccgc

SEQ ID NO: 83 - DNA, 48 bp, synthetic construct; identical to SEQ ID NO: 32
  source 1..48: mol_type = other DNA

SEQ ID NO: 84 - DNA, 3244 bp, synthetic construct
  source 1..3244: mol_type = other DNA
ccacctgacgtctaagaaaccattattatcatgacattaacctataaaaataggcgtatcacgaggcagaatttcagataaaaaaaatccttagctttcgctaaggatgatttctggaattcgcggccgcatctagagtctcgagttgacagctagctcagtcctaggtataatgctagcctcgaggaaagaggagaaaggtctcaatgcgtaaaggcgaagagctgttcactggtgtcgtccctattctggtggaactggatggtgatgtcaacggtcataagttttccgtgcgtggcgagggtgaaggtgacgcaactaatggtaaactgacgctgaagttcatctgtactactggtaaactgccggtaccttggccgactctggtaacgacgctgacttatggtgttcagtgctttgctcgttatccggaccatatgaagcagcatgacttcttcaagtccgccatgccggaaggctatgtgcaggaacgcacgatttcctttaaggatgacggcacgtacaaaacgcgtgcggaagtgaaatttgaaggcgataccctggtaaaccgcattgagctgaaaggcattgactttaaagaagacggcaatatcctgggccataagctggaatacaattttaacagccacaatgtttacatcaccgccgataaacaaaaaaatggcattaaagcgaattttaaaattcgccacaacgtggaggatggcagcgtgcagctggctgatcactaccagcaaaacactccaatcggtgatggtcctgttctgctgccagacaatcactatctgagcacgcaaagcgttctgtctaaagatccgaacgagaaacgcgatcatatggttctgctggagttcgtaaccgcagcgggcatcgcgcatggtatggatgaactgtacagatgataacgctgatagtgctagtgtagatcgctactagagccaggcatcaaataaaacgaaaggctcagtcgaaagactgggcctttcgttttatctgttgtttgtcggtgaacgctctctactagagtcacactggctcaccttcgggtgggcctttctgcgtttatatactagaagcggccgctgcaggaattcaaaaaaagcaccgactcggtgccactttttcaagttgataacggactagccttattttaacttgctatttctagctctaaaacctgaaaccgctgcggcgatgactagtattatacctaggactgagctagctgtcaaggatccagcatatgcggtgtgaaataccgcacagatgcgtaaggagaaaataccgcatcaggcgctcttccgcttcctcgctcactgactcgctgcgctcggtcgttcggctgcggcgagcggtatcagctcactcaaaggcggtaatacggttatccacagaatcaggggataacgcaggaaagaacatgtgagcaaaaggccagcaaaaggccaggaaccgtaaaaaggccgcgttgctggcgtttttccataggctccgcccccctgacgagcatcacaaaaatcgacgctcaagtcagaggtggcgaaacccgacaggactataaagataccaggcgtttccccctggaagctccctcgtgcgctctcctgttccgaccctgccgcttaccggatacctgtccgcctttctcccttcgggaagcgtggcgctttctcatagctcacgctgtaggtatctcagttcggtgtaggtcgttcgctccaagctgggctgtgtgcacgaaccccccgttcagcccgaccgctgcgccttatccggtaactatcgtcttgagtccaacccggtaagacacgacttatcgccactggcagcagccactggtaacaggattagcagagcgaggtatgtaggcggtgctacagagttcttgaagtggtggcctaactacggctacactagaaggacagtatttggtatctgcgctctgctgaagccagttaccttcggaaaaagagttggtagctcttgatccggcaaacaaaccaccgctggtagcggtggtttttttgtttgcaagcagcagattacgcgcagaaaaaaaggatctcaagaagatcctttgatcttttctacggggtctgacgctcagtggaacgaaaactcacgttaagggattttggtcatgagattatcaaaaaggatcttcacctagatccttttaaattaaaaatgaagttttaaatcaatctaaagtatatatgagtaaacttggtctgacagttaccaatgcttaatcagtgaggcacctatctcagcgatctgtctatttcgttcatccatagttgcctgactccccgtcgtgtagataactacgatacgggagggcttaccatctggccccagtgctgcaatgataccgcgtgacccacgctcaccggctccagatttatcagcaataaaccagccagccggaagggccgagcgcagaagtggtcctgcaactttatccgcctccatccagtctattaattgttgccgggaagctagagtaagtagttcgccagttaatagtttgcgcaacgttgttgccattgctacaggcatcgtggtgtcacgctcgtcgtttggtatggcttcattcagctccggttcccaacgatcaaggcgagttacatgatcccccatgttgtgcaaaaaagcggttagctccttcggtcctccgatcgttgtcagaagtaagttggccgcagtgttatcactcatggttatggcagcactgcataattctcttactgtcatgccatccgtaagatgcttttctgtgactggtgagtactcaaccaagtcattctgagaatagtgtatgcggcgaccgagttgctcttgcccggcgtcaatacgggataataccgcgccacatagcagaactttaaaagtgctcatcattggaaaacgttcttcggggcgaaaactctcaaggatcttaccgctgttgagatccagttcgatgtaacccactcgtgcacccaactgatcttcagcatcttttactttcaccagcgtttctgggtgagcaaaaacaggaaggcaaaatgccgcaaaaaagggaataagggcgacacggaaatgttgaatactcatactcttcctttttcaatattattgaagcatttatcagggttattgtctcatgagcggatacatatttgaatgtatttagaaaaataaacaaataggggttccgcgcacatttccccgaaaagtg

SEQ ID NO: 85 - DNA, 15460 bp, synthetic construct
  source 1..15460: mol_type = other DNA
ctgctcgcgcaggctgggtgccaagctctcgggtaacatcaaggcccgatccttggagcccttgccctcccgcacgatgatcgtgccgtgatcgaaatccagatccttgacccgcagttgcaaaccctcactgatccgcatgcggatcttgctgtaggcataggcttggttatgccggtactgccgggcctcttgcgggattacgaaatcatcctgtggagcttagtaggtttagcaagatggcagcgcctaaatgtagaatgataaaaggattaagagattaatttccctaaaaatgataaaacaagcgttttgaaagcgcttgtttttttggtttgcagtcagagtagaatagaagtatcaaaaaaagcaccgactcggtgccactttttcaagttgataacggactagccttattttaacttgctatgctgttttgaatggttccaacaagattattttataacttttataacaaataatcaaggagaaattcaaagaaatttatcagccataaaacaatacttaatactatagaatgataacaaaataaactactttttaaaagaattttgtgttataatctatttattattaagtattgggtaatattttttgaagagatattttgaaaaagaaaaattaaagcatattaaactaatttcggaggtcattaaaactattattgaaatcatcaaactcattatggatttaatttaaactttttattttaggaggcaaaaatggataagaaatactcaataggcttagatatcggcacaaatagcgtcggatgggcggtgatcactgatgaatataaggttccgtctaaaaagttcaaggttctgggaaatacagaccgccacagtatcaaaaaaaatcttataggggctcttttatttgacagtggagagacagcggaagcgactcgtctcaaacggacagctcgtagaaggtatacacgtcggaagaatcgtatttgttatctacaggagattttttcaaatgagatggcgaaagtagatgatagtttctttcatcgacttgaagagtcttttttggtggaagaagacaagaagcatgaacgtcatcctatttttggaaatatagtagatgaagttgcttatcatgagaaatatccaactatctatcatctgcgaaaaaaattggtagattctactgataaagcggatttgcgcttaatctatttggccttagcgcatatgattaagtttcgtggtcattttttgattgagggagatttaaatcctgataatagtgatgtggacaaactatttatccagttggtacaaacctacaatcaattatttgaagaaaaccctattaacgcaagtggagtagatgctaaagcgattctttctgcacgattgagtaaatcaagacgattagaaaatctcattgctcagctccccggtgagaagaaaaatggcttatttgggaatctcattgctttgtcattgggtttgacccctaattttaaatcaaattttgatttggcagaagatgctaaattacagctttcaaaagatacttacgatgatgatttagataatttattggcgcaaattggagatcaatatgctgatttgtttttggcagctaagaatttatcagatgctattttactttcagatatcctaagagtaaatactgaaataactaaggctcccctatcagcttcaatgattaaacgctacgatgaacatcatcaagacttgactcttttaaaagctttagttcgacaacaacttccagaaaagtataaagaaatcttttttgatcaatcaaaaaacggatatgcaggttatattgatgggggagctagccaagaagaattttataaatttatcaaaccaattttagaaaaaatggatggtactgaggaattattggtgaaactaaatcgtgaagatttgctgcgcaagcaacggacctttgacaacggctctattccccatcaaattcacttgggtgagctgcatgctattttgagaagacaagaagacttttatccatttttaaaagacaatcgtgagaagattgaaaaaatcttgacttttcgaattccttattatgttggtccattggcgcgtggcaatagtcgttttgcatggatgactcggaagtctgaagaaacaattaccccatggaattttgaagaagttgtcgataaaggtgcttcagctcaatcatttattgaacgcatgacaaactttgataaaaatcttccaaatgaaaaagtactaccaaaacatagtttgctttatgagtattttacggtttataacgaattgacaaaggtcaaatatgttactgaaggaatgcgaaaaccagcatttctttcaggtgaacagaagaaagccattgttgatttactcttcaaaacaaatcgaaaagtaaccgttaagcaattaaaagaagattatttcaaaaaaatagaatgttttgatagtgttgaaatttcaggagttgaagatagatttaatgcttcattaggtacctaccatgatttgctaaaaattattaaagataaagattttttggataatgaagaaaatgaagatatcttagaggatattgttttaacattgaccttatttgaagatagggagatgattgaggaaagacttaaaacatatgctcacctctttgatgataaggtgatgaaacagcttaaacgtcgccgttatactggttggggacgtttgtctcgaaaattgattaatggtattagggataagcaatctggcaaaacaatattagattttttgaaatcagatggttttgccaatcgcaattttatgcagctgatccatgatgatagtttgacatttaaagaagacattcaaaaagcacaagtgtctggacaaggcgatagtttacatgaacatattgcaaatttagctggtagccctgctattaaaaaaggtattttacagactgtaaaagttgttgatgaattggtcaaagtaatggggcggcataagccagaaaatatcgttattgaaatggcacgtgaaaatcagacaactcaaaagggccagaaaaattcgcgagagcgtatgaaacgaatcgaagaaggtatcaaagaattaggaagtcagattcttaaagagcatcctgttgaaaatactcaattgcaaaatgaaaagctctatctctattatctccaaaatggaagagacatgtatgtggaccaagaattagatattaatcgtttaagtgattatgatgtcgatcacattgttccacaaagtttccttaaagacgattcaatagacaataaggtcttaacgcgttctgataaaaatcgtggtaaatcggataacgttccaagtgaagaagtagtcaaaaagatgaaaaactattggagacaacttctaaacgccaagttaatcactcaacgtaagtttgataatttaacgaaagctgaacgtggaggtttgagtgaacttgataaagctggttttatcaaacgccaattggttgaaactcgccaaatcactaagcatgtggcacaaattttggatagtcgcatgaatactaaatacgatgaaaatgataaacttattcgagaggttaaagtgattaccttaaaatctaaattagtttctgacttccgaaaagatttccaattctataaagtacgtgagattaacaattaccatcatgcccatgatgcgtatctaaatgccgtcgttggaactgctttgattaagaaatatccaaaacttgaatcggagtttgtctatggtgattataaagtttatgatgttcgtaaaatgattgctaagtctgagcaagaaataggcaaagcaaccgcaaaatatttcttttactctaatatcatgaacttcttcaaaacagaaattacacttgcaaatggagagattcgcaaacgccctctaatcgaaactaatggggaaactggagaaattgtctgggataaagggcgagattttgccacagtgcgcaaagtattgtccatgccccaagtcaatattgtcaagaaaacagaagtacagacaggcggattctccaaggagtcaattttaccaaaaagaaattcggacaagcttattgctcgtaaaaaagactgggatccaaaaaaatatggtggttttgatagtccaacggtagcttattcagtcctagtggttgctaaggtggaaaaagggaaatcgaagaagttaaaatccgttaaagagttactagggatcacaattatggaaagaagttcctttgaaaaaaatccgattgactttttagaagctaaaggatataaggaagttaaaaaagacttaatcattaaactacctaaatatagtctttttgagttagaaaacggtcgtaaacggatgctggctagtgccggagaattacaaaaaggaaatgagctggctctgccaagcaaatatgtgaattttttatatttagctagtcattatgaaaagttgaagggtagtccagaagataacgaacaaaaacaattgtttgtggagcagcataagcattatttagatgagattattgagcaaatcagtgaattttctaagcgtgttattttagcagatgccaatttagataaagttcttagtgcatataacaaacatagagacaaaccaatacgtgaacaagcagaaaatattattcatttatttacgttgacgaatcttggagctcccgctgcttttaaatattttgatacaacaattgatcgtaaacgatatacgtctacaaaagaagttttagatgccactcttatccatcaatccatcactggtctttatgaaacacgcattgatttgagtcagctaggaggtgactgaagtatattttagatgaagattatttcttaataactaaaaatatggtataatactcttaataaatgcagtaatacaggggcttttcaagactgaagtctagctgagacaaatagtgcgattacgaaattttttagacaaaaatagtctacgaggttttagagctatgctgttttgaatggtcccaaaactgcagcgcaatagttggcgaagtaatcgcaacatccgcattaaaatctagcgagggctttactaagctccgcaaaaaaccccgcccctgacagggcggggttttttcgcgcccgatccttggagcccttgccctcccgcacgatgatcgtgccgtgatcgaaatccagatccttgacccgcagttgcaaaccctcactgatccgcatgcttatgacaacttgacggctacatcattcactttttcttcacaaccggcacggaactcgctcgggctggccccggtgcattttttaaatacccgcgagaaatagagttgatcgtcaaaaccaacattgcgaccgacggtggcgataggcatccgggtggtgctcaaaagcagcttcgcctggctgatacgttggtcctcgcgccagcttaagacgctaatccctaactgctggcggaaaagatgtgacagacgcgacggcgacaagcaaacatgctgtgcgacgctggcgatatcaaaattgctgtctgccaggtgatcgctgatgtactgacaagcctcgcgtacccgattatccatcggtggatggagcgactcgttaatcgcttccatgcgccgcagtaacaattgctcaagcagatttatcgccagcagctccgaatagcgcccttccccttgcccggcgttaatgatttgcccaaacaggtcgctgaaatgcggctggtgcgcttcatccgggcgaaagaaccccgtattggcaaatattgacggccagttaagccattcatgccagtaggcgcgcggacgaaagtaaacccactggtgataccattcgcgagcctccggatgacgaccgtagtgatgaatctctcctggcgggaacagcaaaatatcacccggtcggcaaacaaattctcgtccctgatttttcaccaccccctgaccgcgaatggtgagattgagaatataacctttcattcccagcggtcggtcgataaaaaaatcgagataaccgttggcctcaatcggcgttaaacccgccaccagatgggcattaaacgagtatcccggcagcaggggatcattttgcgcttcagccatacttttcatactcccgccattcagagaagaaaccaattgtccatattgcatcagacattgccgtcactgcgtcttttactggctcttctcgctaaccaaaccggtaaccccgcttattaaaagcattctgtaacaaagcgggaccaaagccatgacaaaaacgcgtaacaaaagtgtctataatcacggcagaaaagtccacattgattatttgcacggcgtcacactttgctatgccatagcatttttatccataagattagcggatcctacctgacgctttttatcgcaactctctactgtttctccatgtaggtcgttcgctccaagcgttttagagctagaaatagcaagttaaaataaggctagtccgttatcaacttgaaaaagtggcaccagaccccgttgatgataccgctgccttactgggtgcattagccagtctgaatgacctcgagttttagagctatgctgttttgaatggtcccaaaacttcagcacactgagacttgttgagttccatgttttagagctatgctgttttgaatggactccattcaacattgccgatgataacttgagaaagagggttaataccagcagtcggataccttcctattctttctgttaaagcgttttcatgttataataggcaaaagaagagtagtgtgatcgtccattccgacgtcgagccgttccatacagaagctgggcgaacaaacgatgctcgccttccagaaaaccgaggatgcgaaccacttcatccggggtcagcaccaccggcaagcgccgcgacggccgaggtcttccgatctcctgaagccagggcagatccgtgcacagcaccttgccgtagaagaacagcaaggccgccaatgcctgacgatgcgtggagaccgaaaccttgcgctcgttcgccagccaggacagaaatgcctcgacttcgctgctgcccaaggttgccgggtgacgcacaccgtggaaacggatgaaggcacgaacccagtggacataagcctgttcggttcgtaagctgtaatgcaagtagcgtatgcgctcacgcaactggtccagaaccttgaccgaacgcagcggtggtaacggcgcagtggcggttttcatggcttgttatgactgtttttttggggtacagtctatgcctcgggcatccaagcagcaagcgcgttacgccgtgggtcgatgtttgatgttatggagcagcaacgatgttacgcagcagggcagtcgccctaaaacaaagttaaacatcatgagggaagcggtgatcgccgaagtatcgactcaactatcagaggtagttggcgtcatcgagcgccatctcgaaccgacgttgctggccgtacatttgtacggctccgcagtggatggcggcctgaagccacacagtgatattgatttgctggttacggtgaccgtaaggcttgatgaaacaacgcggcgagctttgatcaacgaccttttggaaacttcggcttcccctggagagagcgagattctccgcgctgtagaagtcaccattgttgtgcacgacgacatcattccgtggcgttatccagctaagcgcgaactgcaatttggagaatggcagcgcaatgacattcttgcaggtatcttcgagccagccacgatcgacattgatctggctatcttgctgacaaaagcaagagaacatagcgttgccttggtaggtccagcggcggaggaactctttgatccggttcctgaacaggatctatttgaggcgctaaatgaaaccttaacgctatggaactcgccgcccgactgggctggcgatgagcgaaatgtagtgcttacgttgtcccgcatttggtacagcgcagtaaccggcaaaatcgcgccgaaggatgtcgctgcctactgggcaatggagcgcctgccggcccagtatcagcccgtcatacttgaagctagacaggcttatcttggacaagaagaagatcgcttggcctcgcgcgcagatcagttggaagaatttgtccactacgtgaaaggcgagatcaccaaggtagtcggcaaataatgtctaacaattcgttcaagccgacgccgcttcgcggcgcggcttaactcaagcgttagatgcactaagcacataattgctcacagccaaactatcaggtcaagtctgcttttattatttttaagcgtgcataataagccctacacaaattgggagatatatcatgaaaggctggctttttcttgttatcgcaatagttggcgaagtaatcgcaacatccgcattaaaatctagcgagggctttactaagctcctgcagagatctgaattccctagagagacgaaagtgattgcgcctacccggatattatcgtgaggatgcgtcatcgccattgctccccaaatacaaaaccaatttcagccagtgcctcgtccattttttcgatgaactccggcacgatctcgtcaaaactcgccatgtacttttcatcccgctcaatcacgacataatgcaggccttcacgcttcatacgcgggtcatagttggcaaagtaccaggcattttttcgcgtcacccacatgctgtactgcacctgggccatgtaagctgactttatggcctcgaaaccaccgagccggaacttcatgaaatcccgggaggtaaacgggcatttcagttcaaggccgttgccgtcactgcataaaccatcgggagagcaggcggtacgcatactttcgtcgcgatagatgatcggggattcagtaacattcacgccggaagtgaattcaaacagggttctggcgtcgttctcgtactgttttccccaggccagtgctttagcgttaacttccggagccacaccggtgcaaacctcagcaagcagggtgtggaagtaggacattttcatgtcaggccacttctttccggagcggggttttgctatcacgttgtgaacttctgaagcggtgatgacgccgagccgtaatttgtgccacgcatcttccccctgttcgacagctctcacatcgatcccggtacgctgcaggataatgtccggtgtcatgctgccaccttctgctctgcggctttctgtttcaggaatccaagagcttttactgcttcggcctgtgtcagttctgacgatgcacgaatgtcgcggcgaaatatctgggaacagagcggcaataagtcgtcatcccatgttttatccagggcgatcagcagagtgttaatctcctgcatggtttcatcgttaaccggagtgatgtcgcgttccggctgacgttctgcagtgtatgcagtattttcgacaatgcgctcggcttcatccttgtcatagataccagcaaatccgaaggccagacgggcacactgaatcatggctttatgacgtaacatccgtttgggatgcgactgccacggccccgtgatttctctgccttcgcgagttttgaatggttcgcggcggcattcatccatccattcggtaacgcagatcggatgattacggtccttgcggtaaatccggcatgtacaggattcattgtcctgctcaaagtccatgccatcaaactgctggttttcattgatgatgcgggaccagccatcaacgcccaccaccggaacgatgccattctgcttatcaggaaaggcgtaaatttctttcgtccacggattaaggccgtactggttggcaacgatcagtaatgcgatgaactgcgcatcgctggcatcacctttaaatgccgtctggcgaagagtggtgatcagttcctgtgggtcgacagaatccatgccgacacgttcagccagcttcccagccagcgttgcgagtgcagtactcattcgttttatacctctgaatcaatatcaacctggtggtgagcaatggtttcaaccatgtaccggatgtgttctgccatgcgctcctgaaactcaacatcgtcatcaaacgcacgggtaatggattttttgctggccccgtggcgttgcaaatgatcgatgcatagcgattcaaacaggtgctggggcaggcctttttccatgtcgtctgccagttctgcctctttctcttcacgggcgagctgctggtagtgacgcgcccagctctgagcctcaagacgatcctgaatgtaataagcgttcatggctgaactcctgaaatagctgtgaaaatatcgcccgcgaaatgccgggctgattaggaaaacaggaaagggggttagtgaatgcttttgcttgatctcagtttcagtattaatatccattttttataagcgtcgactgtttcctgtgtgaaattgttatccgctcacaattccacacattatacgagccggaagcataaagtgtaaagcctggggtgcctaatgagtgagaattcggatctcgacgggatgttgattctgtcatggcatatccttacaacttaaaaaagcaaaagggccgcagatgcgacccttgtgtatcaaacaagacgattaaaaatcttcgttagtttctgctacgccttcgctatcatctacagagaaatccggcgttgagttcgggttgctcagcagcaactcacgtactttcttctcgatctctttcgcggtttccgggttatctttcagccaggcagtcgcattcgctttaccctgaccgatcttctcacctttgtagctgtaccacgcgcctgctttctcgatcagcttctcttttacgcccaggtcaaccagttcgccgtagaagttgataccttcgccgtagaggatctggaattcagcctgtttaaacggcgcagcgattttgttcttcaccactttcacgcgggtttcgctacccaccacgttttcgccctctttcaccgcgccgatacgacggatgtcgagacgaacagaggcgtagaatttcagcgcgttaccaccggtagtggtttccgggttaccgaacatcacaccaattttcatacggatctggttgatgaagatcagcagcgtgttggactgcttcaggttacccgccagcttacgcatcgcctggctcatcatacgtgccgcaaggcccatgtgagagtcgccgatttcgccttcgatttccgctttcggcgtcagtgccgccacggagtcaacgacgataacgtctactgcgccagaacgcgccagggcgtcacagatttccagtgcctgctcgccggtgtccggctgggagcacagcaggttgtcgatatcgacgcccagtttacgtgcgtagattgggtccagcgcgtgttcagcatcgataaacgcacaggttttaccttcacgctgcgctgcggcgatcacctgcagcgtcagcgtggttttaccggaagattccggtccgtagatttcgacgatacggcccatcggcagaccacctgccccaagcgcgatatccagtgaaagcgaaccggtagagatggtttccacatccatggaacggtcttcacccaggcgcatgatggagcctttaccaaattgtttctcaatctggcccagtgctgccgccaacgctttctgtttgttttcgtcgatagccatttttactcctgtcatgccgggtaataccggatagtcaatatgttctgttgaagcaattatactgtatgctcatacagtatcaagtgttttgtagaaattgttgccacaaggtctgcaatgcatacgcagtagcctgacgacgcaccgcatcacggtcgccgctgaagcatcccgccgggtaatgccttcaccgcgggcagtggcaaaagcaaaccagacggtgccgacaggcttctctagatccgcctacctttcacgagttgcgcagtttgtctgcaagactctatgagaagcagataagcgataagtttgctcaacatcttctcgggcataagtcggacaccatggcatcacagtatcgtgatgacagaggcagggagtgggacaaaattgaaatcaaataatgattttattttgactgatagtgacctgttcgttgcaacaaattgataagcaatgccaagcttggcactggctgatcagctagctcactgcccgctttccagtcgggaaacctgtcgtgccagctgcattaatgaatcggccaacgcgcggggagaggcggtttgcgtattgggcgccagggtggtttttcttttcaccagtgagacgggcaacagctgattgcccttcaccgcctggccctgagagagttgcagcaagcggtccacgctggtttgccccagcaggcgaaaatcctgtttgatggtggttaacggcgggatataacatgagctgtcttcggtatcgtcgtatcccactaccgagatatccgcaccaacgcgcagcccggactcggtaatggcgcgcattgcgcccagcgccatctgatcgttggcaaccagcatcgcagtgggaacgatgccctcattcagcatttgcatggtttgttgaaaaccggacatggcactccagtcgccttcccgttccgctatcggctgaatttgattgcgagtgagatatttatgccagccagccagacgcagacgcgccgagacagaacttaatgggcccgctaacagcgcgatttgctggtgacccaatgcgaccagatgctccacgcccagtcgcgtaccgtcttcatgggagaaaataatactgttgatgggtgtctggtcagagacatcaagaaataacgccggaacattagtgcaggcagcttccacagcaatggcatcctggtcatccagcggatagttaatgatcagcccactgacgcgttgcgcgagaagattgtgcaccgccgctttacaggcttcgacgccgcttcgttctaccatcgacaccaccacgctggcacccagttgatcggcgcgagatttaatcgccgcgacaatttgcgacggcgcgtgcagggccagactggaggtggcaacgccaatcagcaacgactgtttgcccgccagttgttgtgccacgcggttgggaatgtaattcagctccgccatcgccgcttccactttttcccgcgttttcgcagaaacgtggctggcctggttcaccacgcgggaaacggtctgataagagacaccggcatactctgcgacatcgtataacgttactggtttcacattcaccaccctgaattgactctcttccgggcgctatcatgccataccgcgaaaggttttgcaccattcgatgctagcccatgggtatggacagttttccctttgatatgtaacggtgaacagttgttctacttttgtttgttagtcttgatgcttcactgatagatacaagagccataagaacctcagatccttccgtatttagccagtatgttctctagtgtggttcgttgtttttgcgtgagccatgagaacgaaccattgagatcatacttactttgcatgtcactcaaaaattttgcctcaaaactggtgagctgaatttttgcagttaaagcatcgtgtagtgtttttcttagtccgttacgtaggtaggaatctgatgtaatggttgttggtattttgtcaccattcatttttatctggttgttctcaagttcggttacgagatccatttgtctatctagttcaacttggaaaatcaacgtatcagtcgggcggcctcgcttatcaaccaccaatttcatattgctgtaagtgtttaaatctttacttattggtttcaaaacccattggttaagccttttaaactcatggtagttattttcaagcattaacatgaacttaaattcatcaaggctaatctctatatttgccttgtgagttttcttttgtgttagttcttttaataaccactcataaatcctcatagagtatttgttttcaaaagacttaacatgttccagattatattttatgaatttttttaactggaaaagataaggcaatatctcttcactaaaaactaattctaatttttcgcttgagaacttggcatagtttgtccactggaaaatctcaaagcctttaaccaaaggattcctgatttccacagttctcgtcatcagctctctggttgctttagctaatacaccataagcattttccctactgatgttcatcatctgagcgtattggttataagtgaacgataccgtccgttctttccttgtagggttttcaatcgtggggttgagtagtgccacacagcataaaattagcttggtttcatgctccgttaagtcatagcgactaatcgctagttcatttgctttgaaaacaactaattcagacatacatctcaattggtctaggtgattttaatcactataccaattgagatgggctagtcaatgataattactagtccttttcctttgagttgtgggtatctgtaaattctgctagacctttgctggaaaacttgtaaattctgctagaccctctgtaaattccgctagacctttgtgtgttttttttgtttatattcaagtggttataatttatagaataaagaaagaataaaaaaagataaaaagaatagatcccagccctgtgtataactcactactttagtcagttccgcagtattacaaaaggatgtcgcaaacgctgtttgctcctctacaaaacagaccttaaaaccctaaaggcttaagtagcaccctcgcaagctcggttgcggccgcaatcgggcaaatcgctgaatattccttttgtctccgaccatcaggcacctgagtcgctgtctttttcgtgacattcagttcgctgcgctcacggctctggcagtgaatgggggtaaatggcactacaggcgccttttatggattcatgcaaggaaactacccataatacaagaaaagcccgtcacgggcttctcagggcgttttatggcgggtctgctatgtggtgctatctgactttttgctgttcagcagttcctgccctctgattttccagtctgaccacttcggattatcccgtgacaggtcattcagactggctaatgcacccagtaaggcagcggtatcatcaacggggtctgacgctcagtggaacgaaaactcacgttaagggattttggtcatgagattatcaaaaaggatcttcacctagatccttttaaattaaaaatgaagttttaaatcaatctaaagtatatatgagtaaacttggtctgacagttaccaatgcttaatcagtgaggcacctatctcagcgatctgtctatttcgttcatccatagttgcctgactccccgtcgtgtagataactacgatacgggagggcttaccatctggccccagtgctgcaatgataccgcgagacccacgctcaccggctccagatttatcagcaataaaccagccagccg

SEQ ID NO: 86 - DNA, 5260 bp, synthetic construct
  source 1..5260: mol_type = other DNA
gacgtcccatggctcgagcatgcgagagtagggaactgccaggcatcaaataaaatgaaaggctcagtcgaaagactgggcctttcgttttatctgttgtttgtcggtgaacgctctcctgagtaggacaaatccgccgggagcggatttgaacgttgcgaagcaacggcccggagggtggcgggcaggacgcccgccataaactgccaggcatcaaattaagcagaaggccatcctgacggatggcctttttgcgtggccagtgccaagcttgcatgcagattgcagcattacacgtcttgagcgattgtgtaggctggagctgcttcgaagttcctatactttctagagaataggaacttcggaataggaactaaggaggatattcatatggaccatggctaattcccaggtaccagttgttcttattggtggtgttgctttatggttgcatcgtagtaaatggttgtaacaaaagcaatttttccggctgtctgtatacaaaaacgccgtaaagtttgagcgaagtcaataaactctctacccattcagggcaatatctctcttggatccaaagtgaactctagaaataattttgtttaactttaagaaggagatatacatatgggcagcagccatcaccatcatcaccacagccaggatccgaattcggtgtttcaaaaagttgacgcctacgctggcgacccgattcttacgcttatggagcgttttaaagaagaccctcgcagcgacaaagtgaatttaagtatcggtctgtactacaacgaagacggaattattccacaactgcaagccgtggcggaggcggaagcgcgcctgaatgcgcagcctcatggcgcttcgctttatttaccgatggaagggcttaactgctatcgccatgccattgcgccgctgctgtttggtgcggaccatccggtactgaaacaacagcgcgtagcaaccattcaaacccttggcggctccggggcattgaaagtgggcgcggatttcctgaaacgctacttcccggaatcaggcgtctgggtcagcgatcctacctgggaaaaccacgtagcaatattcgccggggctggattcgaagtgagtacttacccctggtatgacgaagcgactaacggcgtgcgctttaatgacctgttggcgacgctgaaaacattacctgcccgcagtattgtgttgctgcatccatgttgccacaacccaacgggtgccgatctcactaatgatcagtgggatgcggtgattgaaattctcaaagcccgcgagcttattccattcctcgatattgcctatcaaggatttggtgccggtatggaagaggatgcctacgctattcgcgccattgccagcgctggattacccgctctggtgagcaattcgttctcgaaaattttctccctttacggcgagcgcgtcggcggactttctgttatgtgtgaagatgccgaagccgctggccgcgtactggggcaattgaaagcaacagttcgccgcaactactccagcccgccgaattttggtgcgcaggtggtggctgcagtgctgaatgacgaggcattgaaagccagctggctggcggaagtagaagagatgcgtactcgcattctggcaatgcgtcaggaattggtgaaggtattaagcacagagatgccagaacgcaatttcgattatctgcttaatcagcgcggcatgttcagttataccggtttaagtgccgctcaggttgaccgactacgtgaagaatttggtgtctatctcatcgccagcggtcgcatgtgtgtcgccgggttaaatacggcaaatgtacaacgtgtggcaaaggcgtttgctgcggtgatgtaaaagctttaagaaggagatataccatgctttttgataacaaaaatcgcggtgctttaaactcactgaacacaccagatattgcttctttatcaatatcatccatgtcggactatcacgtgtttgattttcccggtaaggacctgcagagagaggaagtgatagatttgctagatcagcaagggtttattcccgacgatttgatcgaacaagaagtagattggttttataactcattgggtattgacgatttgttcttctcgagagaatctccccaattaatctcgaatatcatacattctttgtatgcttcaaagctagatttctttgcgaagtccaaattcaacggaattcagccaaggctattcagcattaaaaacaaaattataactaatgataatcatgccatctttatggaatctaatactggtgtcagcataagcgattctcagcaaaaaaactttaaatttgctagtgacgccgtcggaaacgatactttggagcatggtaaggataccatcaaaaaaaataggattgaaatggatgattcttgtccaccttatgaattagattccgaaattgatgaccttttcctggataacaagtctcaaaaaaactgcagattagtttctttttgggctccagaaagcgaattaaagctaacttttgtttatgagagtgtttaccctaatgatgatccagccggcgtagatatttcctctcaggatttgctgaaaggtgatattgaatcgattagtgataagaccatgtacaaagtttcgtcgaacgaaaataaaaaactatacggtctcttacttaagttggttaaagaaagagaaggtcctgtcattaagactactcgctccgtagaaaataaggatgaaattaggttattagtcgcttacaagcgattcaccactaagcgttattactctgctttgaactctttgttccactattacaagttgaaaccttctaagttctatttagagtcgtttaatgttaaggatgatgacatcattatcttttccgtttatttgaacgagaaccagcaattggaagatgttctacttcacgatgtggaggcagcattgaaacaggttgaaagagaagcttcattgctatacgctatcccaaacaattctttccatgaggtttaccagagacgtcaattctcgcccaaagaagctatatatgctcatattggtgctatattcattaaccattttgttaatcgtttaggctctgattatcaaaaccttttatctcaaatcaccattaagcgtaatgatactactcttttggagattgtagaaaacctaaaaagaaagttaagaaatgaaaccttaactcagcaaactattatcaacatcatgtcgaagcattacactataatttccaagttgtataaaaattttgctcaaattcactattatcataatagtactaaagatatggagaagacattatcttttcaaagactggaaaaagtggagccttttaagaatgaccaagagttcgaagcttacttgaataaattcattccaaatgattcacctgatttgttgatcctgaaaacactgaacatcttcaacaagtctattttgaagacaaatttctttattacaagaaaagtagcaatatcattcagattagatccttccctggtgatgacaaaattcgaatatccagagacaccctatggtatattttttgtcgttggtaatactttcaaagggttccatatcaggttcagagatatcgcaaggggcggtattcgtatagtctgttccaggaatcaggatatttatgatttgaattccaagaacgttattgatgagaactatcaattggcctctactcagcaacgtaaaaataaggatattccagagggtggctctaaaggtgtcatcttattgaacccaggattggtagaacatgaccagacatttgtcgccttttcccaatatgtggatgcaatgattgacattctaatcaacgatccattaaaggaaaactatgtcaaccttttaccaaaggaggaaatattattttttggcccagatgaaggaactgctggtttcgtggattgggcaactaaccatgctcgtgtgaggaactgcccatggtggaaatcatttttgactggaaaatccccatctttgggtggtattccccatgacgaatatggtatgacttctctgggtgttcgtgcttatgttaataaaatttacgaaactttaaacttgacaaattctactgtttacaaattccaaactggtggtccggatggtgatttgggatccaatgaaattcttttatcttcgccaaacgaatgttatttggcaattctggacggttcaggtgtcctgtgtgatcctaaaggtttagataaagatgaattatgccgcttggcacatgaaaggaaaatgatttccgatttcgacacttccaaattatcaaacaacggattttttgtttctgtggatgcaatggatatcatgctaccaaatggtacaattgtagctaacggcacaaccttcagaaacacctttcatactcaaattttcaaatttgtggatcatgtcgacatttttgttccatgcggtggtagaccaaactcaattactctaaataatctacattattttgttgacgaaaagactgggaaatgtaaaattccatatattgtggagggtgccaatctatttataacgcaacctgctaaaaatgctttggaggaacatggctgtattctgttcaaagatgcttctgcaaacaaaggtggtgtcacatcttcatcaatggaagtgttggcctcactagcgcttaacgataacgacttcgtgcacaaatttattggagatgttagtggtgagaggtctgcgttgtacaagtcgtacgttgtagaagtgcagtcaagaattcagaaaaatgctgaattagagtttggtcagttatggaatttgaatcaactaaatggaacccacatttcagaaatttcaaaccaattgtccttcactataaacaaattgaacgacgatctagttgcttctcaagagttgtggctcaatgatctaaaattaagaaactacctattgttggataaaataattccaaaaattctgattgatgttgctgggcctcagtccgtattggaaaacattccagagagctatttgaaagttcttctgtcgagttacttatcaagcacttttgtttaccagaacggtatcgatgttaacattggaaaattcttggaatttattggtgggttaaaaagagaagcggaggcaagtgcttgataaggtaccctgcagactagtgctattcctgccctttggtcgaaaaaaaaagcccgcactgtcaggtgcgggcttttttctgtgtttcctgc

SEQ ID NO: 87 - DNA, 3778 bp, synthetic construct
  source 1..3778: mol_type = other DNA
gacgtcccatggctcgagcatgcgagagtagggaactgccaggcatcaaataaaatgaaaggctcagtcgaaagactgggcctttcgttttatctgttgtttgtcggtgaacgctctcctgagtaggacaaatccgccgggagcggatttgaacgttgcgaagcaacggcccggagggtggcgggcaggacgcccgccataaactgccaggcatcaaattaagcagaaggccatcctgacggatggcctttttgcgtggccagtgccaagcttgcatgcagattgcagcattacacgtcttgagcgattgtgtaggctggagctgcttcgaagttcctatactttctagagaataggaacttcggaataggaactaaggaggatattcatatggaccatggctaattcccaggtaccagttgttcttattggtggtgttgctttatggttgcatcgtagtaaatggttgtaacaaaagcaatttttccggctgtctgtatacaaaaacgccgtaaagtttgagcgaagtcaataaactctctacccattcagggcaatatctctcttggatccaaagtgaactctagaaataattttgtttaactttaagaaggagatatacatatggcacctgttacaattgaaaagttcgtaaatcaagaagaacgacaccttgtttccaaccgatcagcaacaattccgtttggtgaatacatatttaaaagattgttgtccatcgatacgaaatcagttttcggtgttcctggtgacttcaacttatctctattagaatatctctattcacctagtgttgaatcagctggcctaagatgggtcggcacgtgtaatgaactgaacgccgcttatgcggccgacggatattcccgttactctaataagattggctgtttaataaccacgtatggcgttggtgaattaagcgccttgaacggtatagccggttcgttcgctgaaaatgtcaaagttttgcacattgttggtgtggccaagtccatagattcgcgttcaagtaactttagtgatcggaacctacatcatttggtcccacagctacatgattcaaattttaaagggccaaatcataaagtatatcatgatatggtaaaagatagagtcgcttgctcggtagcctacttggaggatattgaaactgcatgtgaccaagtcgataatgttatccgcgatatttacaagtattctaaacctggttatatttttgttcctgcagattttgcggatatgtctgttacatgtgataatttggttaatgttccacgtatatctcaacaagattgtatagtatacccttctgaaaaccaattgtctgacataatcaacaagattactagttggatatattccagtaaaacacctgcgatccttggagacgtactgactgataggtatggtgtgagtaactttttgaacaagcttatctgcaaaactgggatttggaatttttccactgttatgggaaaatctgtaattgatgagtcaaacccaacttatatgggtcaatataatggtaaagaaggtttaaaacaagtctatgaacattttgaactgtgcgacttggtcttgcattttggagtcgacatcaatgaaattaataatgggcattatacttttacttataaaccaaatgctaaaatcattcaatttcatccgaattatattcgccttgtggacactaggcagggcaatgagcaaatgttcaaaggaatcaattttgcccctattttaaaagaactatacaagcgcattgacgtttctaaactttctttgcaatatgattcaaatgtaactcaatatacgaacgaaacaatgcggttagaagatcctaccaatggacaatcaagcattattacacaagttcacttacaaaagacgatgcctaaatttttgaaccctggtgatgttgtcgtttgtgaaacaggctcttttcaattctctgttcgtgatttcgcgtttccttcgcaattaaaatatatatcgcaaggatttttcctttccattggcatggcccttcctgccgccctaggtgttggaattgccatgcaagaccactcaaacgctcacatcaatggtggcaacgtaaaagaggactataagccaagattaattttgtttgaaggtgacggtgcagcacagatgacaatccaagaactgagcaccattctgaagtgcaatattccactagaagttatcatttggaacaataacggctacactattgaaagagccatcatgggccctaccaggtcgtataacgacgttatgtcttggaaatggaccaaactatttgaagcattcggagacttcgacggaaagtatactaatagcactctcattcaatgtccctctaaattagcactgaaattggaggagcttaagaattcaaacaaaagaagcgggatagaacttttagaagtcaaattaggcgaattggatttccccgaacagctaaagtgcatggttgaagcagcggcacttaaaagaaataaaaaataggagctctaagaaggagatataccatgaagatcaaagctgttggtgcatattccgctaaacaaccacttgaaccgatggatatcacccggcgtgaaccgggaccgaatgatgtcaaaatcgaaatcgcttactgtggcgtttgccattccgatctccaccaggtccgttccgagtgggcggggacggtttacccctgcgtgccgggtcatgaaattgtggggcgtgtggtagccgttggtgatcaggtagaaaaatatgcgccgggcgatctggtcggtgtcggctgcattgtcgacagttgtaaacattgcgaagagtgtgaagacgggttggaaaactactgtgatcacatgaccggcacctataactcgccgacgccggacgaaccgggccatactctgggcggctactcacaacagatcgtcgttcatgagcgatatgttctgcgtattcgtcacccgcaagagcagctggcggcggtggctcctttgttgtgtgcagggatcaccacgtattcgccgctacgtcactggcaggccgggccgggtaaaaaagtgggcgtggtcggcatcggcggtctgggacatatggggattaagctggcccacgcgatgggggcacatgtggtggcatttaccacttctgaggcaaaacgcgaagcggcaaaagccctgggggccgatgaagttgttaactcacgcaatgccgatgagatggcggctcatctgaagagtttcgatttcattttgaatacagtagctgcgccacataatctcgacgattttaccaccttgctgaagcgtgatggcaccatgacgctggttggtgcgcctgcgacaccgcataaatcgccggaagttttcaacctgatcatgaaacgccgtgcgatagccggttctatgattggcggcattccagaaactcaggagatgctcgatttttgcgccgaacatggcatcgtggctgatatagagatgattcgggccgatcaaattaatgaagcctatgagcgaatgctgcgcggtgatgtgaaatatcgttttgttatcgataatcgcacactaacagactgaggtaccctcgagtctggtaaagaaaccgctgctgcgaaatttgaacgccagcacatggactcgtctactagcgcagcttaataaggtaccctgcagactagtgctattcctgccctttggtcgaaaaaaaaagcccgcactgtcaggtgcgggcttttttctgtgtttcctgc

SEQ ID NO: 88 - DNA, 2030 bp, synthetic construct
  source 1..2030: mol_type = other DNA
gacgtcccatggctcgagcatgcgagagtagggaactgccaggcatcaaataaaatgaaaggctcagtcgaaagactgggcctttcgttttatctgttgtttgtcggtgaacgctctcctgagtaggacaaatccgccgggagcggatttgaacgttgcgaagcaacggcccggagggtggcgggcaggacgcccgccataaactgccaggcatcaaattaagcagaaggccatcctgacggatggcctttttgcgtggccagtgccaagcttgcatgcagattgcagcattacacgtcttgagcgattgtgtaggctggagctgcttcgaagttcctatactttctagagaataggaacttcggaataggaactaaggaggatattcatatggaccatggctaattcccaggtaccagttgttcttattggtggtgttgctttatggttgcatcgtagtaaatggttgtaacaaaagcaatttttccggctgtctgtatacaaaaacgccgtaaagtttgagcgaagtcaataaactctctacccattcagggcaatatctctcttggatccaaagtgaactctagaaataattttgtttaactttaagaaggagatatacataagctttaagaaggagatataccatgaaaaacgcgtcaaccgtatcggaagatactgcgtcgaatcaagagccgacgcttcatcgcggattacataaccgtcatattcaactgattgcgctgggtggcgcaattggtactggtctgtttcttggcattggcccggcgattcagatggcgggtccggctgtattgctgggctacggcgtcgccgggatcatcgctttcctgattatgcgccagctcggcgagatggtggtcgaagagccggtatccggttcatttgcccactttgcctataaatactggggaccgtttgcgggcttcctctctggctggaactactgggtaatgttcgtgctggtgggaatggcagagctgaccgctgcgggcatctatatgcagtactggttcccggatgttccaacgtggatttgggctgccgccttctttattatcatcaacgccgttaacctggtgaacgtgcgcttatatggcgaaaccgagttctggtttgcgctgattaaagtgctggcgatcatcggtatgatcggctttggcctgtggctgctgttttctgggcacggcggtgagaaagccagtatcaataacctctggcgctacggcggtttctttgccaccggctggaatggattgattttgtcgctggcggtaattatgttctccttcggcggtctggagctgattgggattactgcggctgaagcgcgcgatccggaaaaaagcatccctaaagcagtgaatcaggtggtgtatcgcatcctgctgttttatatcggttcactggtggttttactggcgctctacccgtgggtggaagtgaaatccaacagtagcccgtttgtgatgattttccataatctcgacagcaacgtggtagcttctgcgctgaacttcgtcattctggtggcatcgctgtcggtgtataacagcggggtttactctaacagccgcatgctgtttggcctttctgtgcagggtaatgcgccaaagtttttgactcgcgtcagccgtcgcggcgtgccgattaactcgctgatgctttccggagcgatcacttcgctggtggtgttaatcaactatctgctgccgcaaaaagcgtttggtctgctgatggcgctggtggtagcaacgctgctgttgaactggattatgatctgcctggcgcatctgcgttttcgtgcagcgatgcgtcgtcaggggcgtgaaacacagtttaaggcgctgctctatccgttcggcaactatctttgcatcgccttcctcggcatgattttgctgctgatgtgcacgatggatgatatgcgcttgtcagcgattctgctgccggtgtggattgtgttcctgtttgtggcgtttaaaacattgcgtaggaaagtgaattaa

SEQ ID NO: 89 - protein, 473 aa, synthetic construct
MNISRRKLLLGVGAAGVLAGGAALVPMVRRDGKFVEAKSRASFVEGTQGALPKEADVVIIGAGIQGIMTAINLAERGMSVTILEKGQIAGEQSGRAYSQIISYQTSPEIFPLHHYGKILWRGMNEKIGADTSYRTQGRVEALADEKALDKAQAWIKTAKEAAGFDTPLNTRIIKGEELSNRLVGAQTPWTVAAFEEDSGSVDPETGTPALARYAKQIGVKIYTNCAVRGIETAGGKISDVVSEKGAIKTSQVVLAGGIWSRLFMGNMGIDIPTLNVYLSQQRVSGVPGAPRGNVHLPNGIHFREQADGTYAVAPRIFTSSIVKDSFLLGPKFMHLLGGGELPLEFSIGEDLFNSFKMPTSWNLDEKTPFEQFRVATATQNTQHLDAVFQRMKTEFPVFEKSEVVERWGAVVSPTFDELPIISEVKEYPGLVINTATVWGMTEGPAAGEVTADIVMGKKPVIDPTPFSLDRFKK

SEQ ID NO: 90 - DNA, 1503 bp, synthetic construct
  source 1..1503: mol_type = other DNA
atgactttacctgaatcaaaagacttttcttacttgttttcggatgaaaccaatgctcgtaaaccatccccattgaaaacctgcatccatcttttccaagatcctaacattatctttttgggtggtggcctgccattaaaagattatttcccatgggataatctatctgtagattcacccaagcctccttttccccagggtattggagctccaattgacgagcagaattgcataaaatacaccgtcaacaaagattacgctgataaaagtgccaatccttccaacgatattcctttgtcaagagctttgcaatacgggttcagtgctggtcaacctgaactattaaacttcattagagatcataccaagattatccacgatttgaagtataaggactgggacgttttagccactgcaggtaacacaaatgcctgggaatctactttaagagtcttttgtaaccgaggtgatgtcatcttagttgaggcacattctttttcctcttcattggcttctgcagaggctcaaggtgtcattaccttccccgtgccaattgacgctgatggtatcattcctgaaaaattagctaaagtcatggaaaactggacacctggtgctcctaaaccaaagttgttatacactattccaacgggccaaaatccaactggtacttccattgcagaccatagaaaggaggcaatttacaagatcgctcaaaagtacgacttcctaattgtggaagatgaaccttattatttcttacaaatgaatccctacatcaaagacttgaaggaaagagagaaggcacaaagttctccaaagcaggaccatgacgaatttttgaagtccttggcaaacactttcctttccttggatacagaaggccgtgttattagaatggattccttttcaaaagttttggccccagggacaagattgggttggattactggttcatccaaaatcttgaagccttacttgagtttgcatgaaatgacgattcaagccccagcaggttttacacaagttttggtcaacgctacgctatccaggtggggtcaaaagggttacttggactggttgcttggcctgcgtcatgaatacactttgaaacgtgactgtgccatcgatgccctttacaagtatctaccacaatctgatgctttcgtgatcaatcctccaattgcaggtatgtttttcaccgtgaacattgacgcatctgtccaccctgagtttaaaacaaaatacaactcagacccttaccagctagaacagagtctttaccacaaagtggttgaacgtggtgttttagtggttcccggttcttggttcaagagtgagggtgagacggaacctcctcaacccgctgaatctaaagaagtcagtaatccaaacataattttcttcagaggtacctatgcagctgtctctcctgagaaactgactgaaggtctgaagagattaggtgatactttatacgaagaatttggtatttccaaatag

SEQ ID NO: 91 - DNA, 1422 bp, synthetic construct
  source 1..1422: mol_type = other DNA
atgaacatttcaaggagaaagctacttttaggtgttggtgctgcgggcgttttagcaggtggtgcggctttagttccaatggttcgccgtgacggcaaatttgtggaagctaaatcaagagcatcatttgttgaaggtacgcaaggggctcttcctaaagaagcagatgtagtgattattggtgccggtattcaagggatcatgaccgctattaaccttgctgaacgtggtatgagtgtcactatcttagaaaagggtcagattgccggtgagcaatcaggccgtgcatacagccaaattattagttaccaaacatcgccagaaatcttcccattacaccattatgggaaaatattatggcgtggcatgaatgagaaaattggtgcggataccagttatcgtactcaaggtcgtgtagaagcgctggcagatgaaaaagcattagataaagctcaagcgtggatcaaaacagctaaagaagcggcaggttttgatacaccattaaatactcgcatcattaaaggtgaagagctatcaaatcgcttagtcggtgctcaaacgccatggactgttgctgcatttgaagaagattcaggctctgttgatcctgaaacaggcacacctgcactcgctcgttatgccaaacaaatcggtgtgaaaatttataccaactgtgcagtaagaggtattgaaactgcgggtggtaaaatctctgatgtggtgagtgagaaaggggcgattaaaacgtctcaagttgtactcgctgggggtatctggtcgcgtttatttatgggcaatatgggtattgatatcccaacgctcaatgtatatctatcacaacaacgtgtctcaggggttcctggtgcaccacgtggtaatgtgcatttacctaatggtattcatttccgcgaacaagcggatggtacttatgccgttgcaccacgtatctttacgagttcaatagtcaaagatagcttcctgctagggcctaaatttatgcacttattaggtggcggagagttaccgttggaattctctattggtgaagatctatttaattcatttaaaatgccgacctcttggaatttagatgaaaaaacaccattcgaacaattccgagttgccacggcaacacaaaatacgcaacacttagatgctgttttccaaagaatgaaaacagaattcccagtatttgaaaaatcagaagttgttgaacgttggggtgccgttgtgagtccaacatttgatgaattacctatcatttctgaggtcaaagaatacccaggcttagtgattaacacggcaacagtgtggggtatgacagaaggcccggcagcgggtgaagtgaccgctgatattgtcatgggcaagaaacctgttattgatccaacgccgtttagtttggatcgttttaagaagtaa

SEQ ID NO: 92 - DNA, 1140 bp, synthetic construct
  source 1..1140: mol_type = other DNA
atgattttggtaactttagaacagactttacaagacgacaaggcaagtgttttggataaaatggtcgagcatgaacaaattctattttgtcatgataaagcaaccggtcttcaagccatcattgcagtccacgatacgactatgggacctgcactcggtggatgtcgcatggcgccttataaaacgatggatctcgcattaaaagatgttcttcgcctttcaaaagggatgacatataaatgtgcggcagctgatgtagactttggcggcggaaaatccgtcatcatcggagacccgctaaaagataaaacgcctgagaaattccgtgctttcggtcaattcatcgaatcattgaacggacgcttctatacaggtacagacatgggcacaacgcttgaagactttgtgcatgccatgaaagaaacaaactacatcgtgggcaagccggtcgaatatggtggcggtggagactcatcgatccctactgcactcggagtcttctatggcattaaagcgacaaaccagaatctgtttggcgacgacaaagtagaaggccgaaaatacagtatccaaggtcttgggaaagtaggttacaaagtagctgaacatattatcaacgaaggtggaaacgtgatcgtcacagatattaatgagcaagcgattgcagatattcagaagctcggtggaagcgctgtcagggtcgtatcaagtgaggagatttacagtcagcaagcagatgtttttgttccttgtgcatttggtggcgtgatcaatgacgacacgctaaaggtgctgaaagtacgaggaatctccggttcagcaaacaatcagctcgcggaaagccgccatggagagctactacgtgaaaagggtattttgtacgcaccagactatatcgtcaacggcggcggtttaatccaagtggcggatgaattgtacggaacgaatcctgcacgtgtactcgctaaaactgaaaacatctatacctcactgcttgaagtattccatcaggcagaacaggatcatatgacaactgccactgccgcagaccgtatgtgtgaaaagcgtattgcggatgccaagaatcgcaacagcttcttcacacagtcaaaccgaccgaaatggaattttcatcagtaa

SEQ ID NO: 93 - DNA, 1146 bp, synthetic construct
  source 1..1146: mol_type = other DNA
atggcaaaacagcttgaaaagtcatcaaaaattggtaatgaggacgtttttcaaaaaatagcgaatcacgagcagattgtgttctgtaatgatccggtatccggcctgcaagctatcattgctatccacgatacaaccctaggccccgctttaggtggaactcgcatgtatccctataaaaatgtggatgaagctctggaagatgtgcttcgcctgtcagaaggaatgacgtataaatgcgcagccgccgatatcgatttcggcggcgggaaggcggtcattatcggagatccagaaaaggataaatctccggcattgttccgtgcatttggtcaatttgtggaatcactgaatggacgattttacacaggtactgacatggggaccacgatggatgattttgtccatgcacagaaagagacgaatttcattaacggaattcctgagcagtatggtggaagcggcgactcgtcgattccgaccgcccagggagtcatttatgcactgaaggctacaaaccagtatttatttggaagcgatagcctttcaggtaaaacatatgctattcaagggctgggaaaagtagggtataaagtagcggaacagctcttaaaagccggcgccgatttatttgtaacggatatacatgaaaatgtcctcaattccattaagcaaaaatcagaagagcttggcggttcagtgaccattgtaaaaagtgacgatatttacagcgtacaagcggatatatttgttccgtgtgcgatgggtggtattatcaatgataaaaccattcctaagttaaaggtgaaggctgttgtgggatcagccaataaccagctcaaagacctccgccatgcaaatgtactaaacgaaaagggaattctatatgcacccgattatatcgtcaatgccggcggcttgatccaggttgctgacgaactttatgggccgaataaagagcgggtcttgctcaaaacgaaagaaatttaccgttctctgcttgaaatttttaatcaggcagcccttgactgcatcacaacagtggaggccgcaaataggaagtgtcaaaagacgattgagggccagcaaacccgtaatagtttcttttctaggggacgcaggccgaagtggaacataaaagagtaa

SEQ ID NO: 94 - DNA, 1143 bp, synthetic construct
  source 1..1143: mol_type = other DNA
atgagcttagtagaaaaaacatccatcataaaagatttcactctttttgaaaaaatgtctgaacatgaacaagttgttttttgcaacgatccggcgacaggactaagggccattatcgctattcatgacaccacactcggacctgcgctcggcggctgccgcatgcagccttataacagtgtggaagaagcattggaagatgctcttcgcctttccaaaggaatgacttacaaatgcgcggcgtccgatgtcgactttggcggcggaaaagcagtcattatcggtgatccgcagaaagataaatctccagaactgttccgcgcgtttggccaatttgttgattcgcttggcggccgtttctatacaggtactgatatgggaacgaatatggaagatttcattcacgccatgaaagaaacaaactgcattgttggggtgccggaagcttacggcggcggcggagattcctctattccaactgccatgggtgtcctgtacggcattaaagcaaccaacaaaatgttgtttggcaaggacgatcttggcggcgtcacttatgccattcaaggacttggcaaagtaggctacaaagtagcggaagggctgctcgaagaaggtgctcatttatttgtaacggatattaacgagcaaacgttggaggctatccaggaaaaagcaaaaacaacatccggttctgtcacggtagtagcgagcgatgaaatttattcccaggaagccgatgtgttcgttccgtgtgcatttggcggcgttgttaatgatgaaacgatgaagcagttcaaggtgaaagcaatcgccggttcagccaacaatcagctgcttacggaggatcacggcagacaccttgcagacaaaggcattctgtatgctccggattatattgttaactctggcggtctgatccaagtagccgacgaattgtatgaggtgaacaaagaacgcgtgcttgcgaagacgaagcatatttacgacgcaattcttgaagtgtaccagcaagcggaattagatcaaatcaccacaatggaagcagccaacagaatgtgtgagcaaagaatggcggcaagaggccgacgcaacagcttctttacttcttctgttaagccaaaatgggatattcgcaactaa

SEQ ID NO: 95 - DNA, 1650 bp, synthetic construct
  source 1..1650: mol_type = other DNA
atgacaaacacagttattaagtacgttttagaccgattatatgatttaggtatcaaagatatttttggtgttgctggtgattacgccttccctattgaagacactgtttgcaacaaccaacaacaacgttggattggtaactgtaatgaattaaatgcggcatatgctgcagatggctatgctcgaattaaaggaatggcggcattatccactacctttggtgtaggtgaattaagcgcgattaacgctattgccggtgcctatgccgaaaatttaccgattttccatttagttggcatgccagcaagtggcgtacaaaaaagtaaacgtcttgtgcatcatactttaggtaatggtgattttgatgttttttatcagattgctcagcgccttgcttgcgctcatactattttaacacccgaaaattgtgtggaagaaatggagcgcgtaatagaagcagcattaaaagagcgtcgtcctgtttatattggtataccttcagattatgctaatagccaagtagtagcgccgttatctgttaccgcaccacaaaagccaacaagtgataaagcaacattagaaaaagcagtatcagcaatcattgagaaactcacccacagcaataatgtctgtgtattaccaggctttttatctgcacgtttagggttaacagataaaatccagcattttattgataaaacaggtttaccttatgccactatgtttatggataaaagcatattaagtgaatctaacactcaatatgttggtatgtatgacggacaattaatgacaccagaggtcagagaatttgtcgaaagtagtgaatatatattagggatcggtacattactgactgactttaatacaggcagtttcactgctaatataaaatcagaacaatttatcagtatcatgccagactatgttgaaattgattctgtgatctactcctgcgtttatatgacagatattctttctgaattaacccaacgactgccgaataaaacttatcataaaataacagcgaaaggattaggtgaagcggttacatctgataataataaaattacagcacaatatctctatcctcgtttagaacaattctttaagcctaatgatattattattgcagaaacaggaacatcatccatgggattaggcttcgctttattacctgaaggtgcacaatttcataatcaaacactatggggctctattggttgggcaacaccggctgcattaggcgctgcgttagcggcaccagaaaaacgcattattttaattaccggtgaaggctcacatcagttaacagtacaagaaattagtcaatttgttcgtttcggtttaaaacctattattctagtattaaataacgatggttatttaatagagagattattatgtgattaccccgaagcttattataatgatttagctcagtggaactatcatcagttacctcaagcctttggtgcaacagattggtatagtgaaaaagtaactacagcaagtggactagataatgcgttaaataaagccgcactaacaaatagcgcatcttatattgagatagtcacagagcgatatgaggcctctgaattagcgcaaaatttaaaaggatcaaaaagttcattatattcattctaa

SEQ ID NO: 96 - DNA, 1434 bp, synthetic construct
  source 1..1434: mol_type = other DNA
atgaacacagaaaacattgaacaagccatccgtaaaattttgagtgaagaacttagcaatcctcagtcatcaacggccaccaatacgaccgttcccggcaaaaatgggatctttaagacggtcaatgaagccattgcggccacaaaagcggcgcaagaaaactacgccgaccaaccaatctcagttcggaacaaagtgattgatgcgatccgtgagggtttccggccatacattgaggatatggctaagcggattcatgacgaaactggcatgggaacggttagcgcgaaaattgccaaactcaataacgccctttataacacacccggtccagaaattctgcagccagaagccgaaaccggtgacggtggactggttatgtatgaatacgcgccatttggtgtcattggtgccgttggtcctagtaccaacccctctgaaacggtgattgccaatgccatcatgatgttggctggtgggaatacgttgttctttggtgcccatccaggtgctaagaacattacccgttggacgatcgaaaaattaaacgaattggtagctgatgcaactgggttacataacttagtcgtttcactggaaacgccttcaattgaatccgtgcaagaagttatgcaacatcctgacgttgccatgctgtcaatcactggagggcctgctgttgtccaccaagcgcttatcagtggtaagaaggcggttggtgccggtgctggtaacccaccggcaatggtggatgcaactgccaatattgctttagcagcccacaacattgttgattcagcagcctttgataataacattctctgcacggccgaaaaggaagttgtcgttgaagccgctgtcaaggatgaactcatcatgcggatgcaacaagaaggggccttcttggttaccgattctgccgatattgaaaaattagcgcaaatgaccattgggcctaagggcgcaccagatcggaagtttgttggtaaagatgccacttacattttggatcaagcaggaatctcttacaccgggacaccaacactgattattcttgaagcagctaaggatcatccgttagtaacgacagaaatgttgatgccaattttgccagtcgtttgttgccctgactttgatagcgttttagcaacggctacagaagttgaaggtgggttacaccacacggcttccattcattccgagaatttaccacacatcaataaggcagcgcaccggttgaatacgtcaatcttcgtggttaacggcccaacttattgtgggactggtgttgcaacgaatggtgcgcatagtggggcttcagccttaacgattgccacaccaacgggtgaaggaacggcaacgtctaagacttacacgcgccggcgccggcttaactcgccagaagggttctcattacggacttgggaggcttag

SEQ ID NO: 97 - DNA, 3279 bp, synthetic construct
  source 1..3279: mol_type = other DNA
atgctttttgataacaaaaatcgcggtgctttaaactcactgaacacaccagatattgcttctttatcaatatcatccatgtcggactatcacgtgtttgattttcccggtaaggacctgcagagagaggaagtgatagatttgctagatcagcaagggtttattcccgacgatttgatcgaacaagaagtagattggttttataactcattgggtattgacgatttgttcttctcgagagaatctccccaattaatctcgaatatcatacattctttgtatgcttcaaagctagatttctttgcgaagtccaaattcaacggaattcagccaaggctattcagcattaaaaacaaaattataactaatgataatcatgccatctttatggaatctaatactggtgtcagcataagcgattctcagcaaaaaaactttaaatttgctagtgacgccgtcggaaacgatactttggagcatggtaaggataccatcaaaaaaaataggattgaaatggatgattcttgtccaccttatgaattagattccgaaattgatgaccttttcctggataacaagtctcaaaaaaactgcagattagtttctttttgggctccagaaagcgaattaaagctaacttttgtttatgagagtgtttaccctaatgatgatccagccggcgtagatatttcctctcaggatttgctgaaaggtgatattgaatcgattagtgataagaccatgtacaaagtttcgtcgaacgaaaataaaaaactatacggtctcttacttaagttggttaaagaaagagaaggtcctgtcattaagactactcgctccgtagaaaataaggatgaaattaggttattagtcgcttacaagcgattcaccactaagcgttattactctgctttgaactctttgttccactattacaagttgaaaccttctaagttctatttagagtcgtttaatgttaaggatgatgacatcattatcttttccgtttatttgaacgagaaccagcaattggaagatgttctacttcacgatgtggaggcagcattgaaacaggttgaaagagaagcttcattgctatacgctatcccaaacaattctttccatgaggtttaccagagacgtcaattctcgcccaaagaagctatatatgctcatattggtgctatattcattaaccattttgttaatcgtttaggctctgattatcaaaaccttttatctcaaatcaccattaagcgtaatgatactactcttttggagattgtagaaaacctaaaaagaaagttaagaaatgaaaccttaactcagcaaactattatcaacatcatgtcgaagcattacactataatttccaagttgtataaaaattttgctcaaattcactattatcataatagtactaaagatatggagaagacattatcttttcaaagactggaaaaagtggagccttttaagaatgaccaagagttcgaagcttacttgaataaattcattccaaatgattcacctgatttgttgatcctgaaaacactgaacatcttcaacaagtctattttgaagacaaatttctttattacaagaaaagtagcaatatcattcagattagatccttccctggtgatgacaaaattcgaatatccagagacaccctatggtatattttttgtcgttggtaatactttcaaagggttccatatcaggttcagagatatcgcaaggggcggtattcgtatagtctgttccaggaatcaggatatttatgatttgaattccaagaacgttattgatgagaactatcaattggcctctactcagcaacgtaaaaataaggatattccagagggtggctctaaaggtgtcatcttattgaacccaggattggtagaacatgaccagacatttgtcgccttttcccaatatgtggatgcaatgattgacattctaatcaacgatccattaaaggaaaactatgtcaaccttttaccaaaggaggaaatattattttttggcccagatgaaggaactgctggtttcgtggattgggcaactaaccatgctcgtgtgaggaactgcccatggtggaaatcatttttgactggaaaatccccatctttgggtggtattccccatgacgaatatggtatgacttctctgggtgttcgtgcttatgttaataaaatttacgaaactttaaacttgacaaattctactgtttacaaattccaaactggtggtccggatggtgatttgggatccaatgaaattcttttatcttcgccaaacgaatgttatttggcaattctggacggttcaggtgtcctgtgtgatcctaaaggtttagataaagatgaattatgccgcttggcacatgaaaggaaaatgatttccgatttcgacacttccaaattatcaaacaacggattttttgtttctgtggatgcaatggatatcatgctaccaaatggtacaattgtagctaacggcacaaccttcagaaacacctttcatactcaaattttcaaatttgtggatcatgtcgacatttttgttccatgcggtggtagaccaaactcaattactctaaataatctacattattttgttgacgaaaagactgggaaatgtaaaattccatatattgtggagggtgccaatctatttataacgcaacctgctaaaaatgctttggaggaacatggctgtattctgttcaaagatgcttctgcaaacaaaggtggtgtcacatcttcatcaatggaagtgttggcctcactagcgcttaacgataacgacttcgtgcacaaatttattggagatgttagtggtgagaggtctgcgttgtacaagtcgtacgttgtagaagtgcagtcaagaattcagaaaaatgctgaattagagtttggtcagttatggaatttgaatcaactaaatggaacccacatttcagaaatttcaaaccaattgtccttcactataaacaaattgaacgacgatctagttgcttctcaagagttgtggctcaatgatctaaaattaagaaactacctattgttggataaaataattccaaaaattctgattgatgttgctgggcctcagtccgtattggaaaacattccagagagctatttgaaagttcttctgtcgagttacttatcaagcacttttgtttaccagaacggtatcgatgttaacattggaaaattcttggaatttattggtgggttaaaaagagaagcggaggcaagtgcttga

SEQ ID NO: 98 - DNA, 35 bp, synthetic construct
  source 1..35: mol_type = other DNA
ttgacggctagctcagtcctaggtacagtgctagc

SEQ ID NO: 99 - DNA, 44 bp, synthetic construct
  source 1..44: mol_type = other DNA
ttgacaattaatcatccggctcgtataatgtgtggaattgtgag

SEQ ID NO: 100 - DNA, 44 bp, synthetic construct
  source 1..44: mol_type = other DNA
tccctatcagtgatagagattgacatccctatcagtgatagaga

SEQ ID NO: 101 - DNA, 52 bp, synthetic construct
  source 1..52: mol_type = other DNA
attggatccaattgacagctagctcagtcctaggtaccattggatccaatag

SEQ ID NO: 102 - DNA, 255 bp, synthetic construct
  source 1..255: mol_type = other DNA
atggagaaacagtagagagttgcgaaaaaaagcgtcaggctggatccgctaatcttatggataaaaatgctatggcatagcaaagtgtgacgccgtgcaaataatcaatgtggacttttctgccgtgattatagacacttttgttacgcgtttttgtcatggctttggtcccgctttgttacagaatgcttttaataagcggggttaccggttgggttagcgagaagagccagtaaaagacgcagtgacggcaat

SEQ ID NO: 103 - DNA, 735 bp, synthetic construct
  source 1..735: mol_type = other DNA
atggacatgcctcgtattaaaccgggtcagcgtgttatgatggcactgcgtaaaatgattgcaagcggtgaaatcaaaagtggtgaacgtattgcagaaattccgaccgcagcagcactgggtgttagccgtatgccggttcgtatcgcactgcgttcactggaacaagaaggtctggttgttcgtctgggtgcacgtggttatgcagcccgtggtgttagcagcgatcagattcgtgatgcaattgaagttcgtggtgttctggaaggttttgcagcacgtcgtctggcagaacgtggtatgaccgcagaaacccatgcacgttttgttgtactgattgcagaaggtgaagcactgtttgcagccggtcgcctgaatggtgaagatctggatcgttatgccgcatataatcaggcatttcatgataccctggttagcgcagcaggtaatggtgcagttgaaagcgcactggcacgtaatggttttgaaccgtttgcagcagccggtgcactggccctggatctgatggacctgtctgccgaatatgaacatctgctggcagcacatcgtcagcatcaggcagttctggatgcagttagctgtggtgatgccgaaggtgcagaacgtattatgcgtgatcatgcactggcagcaattcgtaatgcaaaagtttttgaagcagcagcaagcgcaggcgcaccgctgggtgcagcatggtcaattcgtgcagattga

SEQ ID NO: 104 - DNA, 5215 bp, synthetic construct
  source 1..5215: mol_type = other DNA
gacgtcccatggctcgagcatgcgagagtagggaactgccaggcatcaaataaaatgaaaggctcagtcgaaagactgggcctttcgttttatctgttgtttgtcggtgaacgctctcctgagtaggacaaatccgccgggagcggatttgaacgttgcgaagcaacggcccggagggtggcgggcaggacgcccgccataaactgccaggcatcaaattaagcagaaggccatcctgacggatggcctttttgcgtggccagtgccaagcttgcatgcagattgcagcattacacgtcttgagcgattgtgtaggctggagctgcttcgaagttcctatactttctagagaataggaacttcggaataggaactaaggaggatattcatatggaccatggctaattcccaggtaccagttgttcttattggtggtgttgctttatggttgcatcgtagtaaatggttgtaacaaaagcaatttttccggctgtctgtatacaaaaacgccgtaaagtttgagcgaagtcaataaactctctacccattcagggcaatatctctcttggatccaaagtgaactctagaaataattttgtttaactttaagaaggagatatacatatggtgtttcaaaaagttgacgcctacgctggcgacccgattcttacgcttatggagcgttttaaagaagaccctcgcagcgacaaagtgaatttaagtatcggtctgtactacaacgaagacggaattattccacaactgcaagccgtggcggaggcggaagcgcgcctgaatgcgcagcctcatggcgcttcgctttatttaccgatggaagggcttaacagctatcgccatgccattgcgccgctgctgtttggtgcggaccatccggtactgaaacaacagcgcgtagcaaccattcaaacccttggcggctccggggcattgaaagtgggcgcggatttcctgaaacgctacttcccggaatcaggcgtctgggtcagcgatcctacctgggaaaaccacgtagcaatattcgccggggctggattcgaagtgagtacttacccctggtatgacgaagcgactaacggcgtgcgctttaatgacctgttggcgacgctgaaaacattacctgcccgcagtattgtgttgctgcatccatgttgccacaacccaacgggtgccgatctcactaatgatcagtgggatgcggtgattgaaattctcaaagcccgcgagcttattccattcctcgatattgcctatcaaggatttggtgccggtatggaagaggatgcctacgctattcgcgccattgccagcgctggattacccgctctggtgagcaattcgttctcgaaaattttctccctttacggcgagcgcgtcggcggactttctgttatgtgtgaagatgccgaagccgctggccgcgtactggggcaattgaaagcaacagttcgccgcaactactccagcccgccgaattttggtgcgcaggtggtggctgcagtgctgaatgacgaggcattgaaagccagctggctggcggaagtagaagagatgcgtactcgcattctggcaatgcgtcaggaattggtgaaggtattaagcacagagatgccagaacgcaatttcgattatctgcttaatcagcgcggcatgttcagttataccggtttaagtgccgctcaggttgaccgactacgtgaagaatttggtgtctatctcatcgccagcggtcgcatgtgtgtcgccgggttaaatacggcaaatgtacaacgtgtggcaaaggcgtttgctgcggtgatgtaaaagctttaagaaggagatataccatgctttttgataacaaaaatcgcggtgctttaaactcactgaacacaccagatattgcttctttatcaatatcatccatgtcggactatcacgtgtttgattttcccggtaaggacctgcagagagaggaagtgatagatttgctagatcagcaagggtttattcccgacgatttgatcgaacaagaagtagattggttttataactcattgggtattgacgatttgttcttctcgagagaatctccccaattaatctcgaatatcatacattctttgtatgcttcaaagctagatttctttgcgaagtccaaattcaacggaattcagccaaggctattcagcattaaaaacaaaattataactaatgataatcatgccatctttatggaatctaatactggtgtcagcataagcgattctcagcaaaaaaactttaaatttgctagtgacgccgtcggaaacgatactttggagcatggtaaggataccatcaaaaaaaataggattgaaatggatgattcttgtccaccttatgaattagattccgaaattgatgaccttttcctggataacaagtctcaaaaaaactgcagattagtttctttttgggctccagaaagcgaattaaagctaacttttgtttatgagagtgtttaccctaatgatgatccagccggcgtagatatttcctctcaggatttgctgaaaggtgatattgaatcgattagtgataagaccatgtacaaagtttcgtcgaacgaaaataaaaaactatacggtctcttacttaagttggttaaagaaagagaaggtcctgtcattaagactactcgctccgtagaaaataaggatgaaattaggttattagtcgcttacaagcgattcaccactaagcgttattactctgctttgaactctttgttccactattacaagttgaaaccttctaagttctatttagagtcgtttaatgttaaggatgatgacatcattatcttttccgtttatttgaacgagaaccagcaattggaagatgttctacttcacgatgtggaggcagcattgaaacaggttgaaagagaagcttcattgctatacgctatcccaaacaattctttccatgaggtttaccagagacgtcaattctcgcccaaagaagctatatatgctcatattggtgctatattcattaaccattttgttaatcgtttaggctctgattatcaaaaccttttatctcaaatcaccattaagcgtaatgatactactcttttggagattgtagaaaacctaaaaagaaagttaagaaatgaaaccttaactcagcaaactattatcaacatcatgtcgaagcattacactataatttccaagttgtataaaaattttgctcaaattcactattatcataatagtactaaagatatggagaagacattatcttttcaaagactggaaaaagtggagccttttaagaatgaccaagagttcgaagcttacttgaataaattcattccaaatgattcacctgatttgttgatcctgaaaacactgaacatcttcaacaagtctattttgaagacaaatttctttattacaagaaaagtagcaatatcattcagattagatccttccctggtgatgacaaaattcgaatatccagagacaccctatggtatattttttgtcgttggtaatactttcaaagggttccatatcaggttcagagatatcgcaaggggcggtattcgtatagtctgttccaggaatcaggatatttatgatttgaattccaagaacgttattgatgagaactatcaattggcctctactcagcaacgtaaaaataaggatattccagagggtggctctaaaggtgtcatcttattgaacccaggattggtagaacatgaccagacatttgtcgccttttcccaatatgtggatgcaatgattgacattctaatcaacgatccattaaaggaaaactatgtcaaccttttaccaaaggaggaaatattattttttggcccagatgaaggaactgctggtttcgtggattgggcaactaaccatgctcgtgtgaggaactgcccatggtggaaatcatttttgactggaaaatccccatctttgggtggtattccccatgacgaatatggtatgacttctctgggtgttcgtgcttatgttaataaaatttacgaaactttaaacttgacaaattctactgtttacaaattccaaactggtggtccggatggtgatttgggatccaatgaaattcttttatcttcgccaaacgaatgttatttggcaattctggacggttcaggtgtcctgtgtgatcctaaaggtttagataaagatgaattatgccgcttggcacatgaaaggaaaatgatttccgatttcgacacttccaaattatcaaacaacggattttttgtttctgtggatgcaatggatatcatgctaccaaatggtacaattgtagctaacggcacaaccttcagaaacacctttcatactcaaattttcaaatttgtggatcatgtcgacatttttgttccatgcggtggtagaccaaactcaattactctaaataatctacattattttgttgacgaaaagactgggaaatgtaaaattccatatattgtggagggtgccaatctatttataacgcaacctgctaaaaatgctttggaggaacatggctgtattctgttcaaagatgcttctgcaaacaaaggtggtgtcacatcttcatcaatggaagtgttggcctcactagcgcttaacgataacgacttcgtgcacaaatttattggagatgttagtggtgagaggtctgcgttgtacaagtcgtacgttgtagaagtgcagtcaagaattcagaaaaatgctgaattagagtttggtcagttatggaatttgaatcaactaaatggaacccacatttcagaaatttcaaaccaattgtccttcactataaacaaattgaacgacgatctagttgcttctcaagagttgtggctcaatgatctaaaattaagaaactacctattgttggataaaataattccaaaaattctgattgatgttgctgggcctcagtccgtattggaaaacattccagagagctatttgaaagttcttctgtcgagttacttatcaagcacttttgtttaccagaacggtatcgatgttaacattggaaaattcttggaatttattggtgggttaaaaagagaagcggaggcaagtgcttgataaggtaccctgcagactagtgctattcctgccctttggtcgaaaaaaaaagcccgcactgtcaggtgcgggcttttttctgtgtttcctgc

SEQ ID NO: 105 - DNA, 3715 bp, synthetic construct
  source 1..3715: mol_type = other DNA
gacgtcccatggctcgagcatgcgagagtagggaactgccaggcatcaaataaaatgaaaggctcagtcgaaagactgggcctttcgttttatctgttgtttgtcggtgaacgctctcctgagtaggacaaatccgccgggagcggatttgaacgttgcgaagcaacggcccggagggtggcgggcaggacgcccgccataaactgccaggcatcaaattaagcagaaggccatcctgacggatggcctttttgcgtggccagtgccaagcttgcatgcagattgcagcattacacgtcttgagcgattgtgtaggctggagctgcttcgaagttcctatactttctagagaataggaacttcggaataggaactaaggaggatattcatatggaccatggctaattcccaggtaccagttgttcttattggtggtgttgctttatggttgcatcgtagtaaatggttgtaacaaaagcaatttttccggctgtctgtatacaaaaacgccgtaaagtttgagcgaagtcaataaactctctacccattcagggcaatatctctcttggatccaaagtgaactctagaaataattttgtttaactttaagaaggagatatacatatggcacctgttacaattgaaaagttcgtaaatcaagaagaacgacaccttgtttccaaccgatcagcaacaattccgtttggtgaatacatatttaaaagattgttgtccatcgatacgaaatcagttttcggtgttcctggtgacttcaacttatctctattagaatatctctattcacctagtgttgaatcagctggcctaagatgggtcggcacgtgtaatgaactgaacgccgcttatgcggccgacggatattcccgttactctaataagattggctgtttaataaccacgtatggcgttggtgaattaagcgccttgaacggtatagccggttcgttcgctgaaaatgtcaaagttttgcacattgttggtgtggccaagtccatagattcgcgttcaagtaactttagtgatcggaacctacatcatttggtcccacagctacatgattcaaattttaaagggccaaatcataaagtatatcatgatatggtaaaagatagagtcgcttgctcggtagcctacttggaggatattgaaactgcatgtgaccaagtcgataatgttatccgcgatatttacaagtattctaaacctggttatatttttgttcctgcagattttgcggatatgtctgttacatgtgataatttggttaatgttccacgtatatctcaacaagattgtatagtatacccttctgaaaaccaattgtctgacataatcaacaagattactagttggatatattccagtaaaacacctgcgatccttggagacgtactgactgataggtatggtgtgagtaactttttgaacaagcttatctgcaaaactgggatttggaatttttccactgttatgggaaaatctgtaattgatgagtcaaacccaacttatatgggtcaatataatggtaaagaaggtttaaaacaagtctatgaacattttgaactgtgcgacttggtcttgcattttggagtcgacatcaatgaaattaataatgggcattatacttttacttataaaccaaatgctaaaatcattcaatttcatccgaattatattcgccttgtggacactaggcagggcaatgagcaaatgttcaaaggaatcaattttgcccctattttaaaagaactatacaagcgcattgacgtttctaaactttctttgcaatatgattcaaatgtaactcaatatacgaacgaaacaatgcggttagaagatcctaccaatggacaatcaagcattattacacaagttcacttacaaaagacgatgcctaaatttttgaaccctggtgatgttgtcgtttgtgaaacaggctcttttcaattctctgttcgtgatttcgcgtttccttcgcaattaaaatatatatcgcaaggatttttcctttccattggcatggcccttcctgccgccctaggtgttggaattgccatgcaagaccactcaaacgctcacatcaatggtggcaacgtaaaagaggactataagccaagattaattttgtttgaaggtgacggtgcagcacagatgacaatccaagaactgagcaccattctgaagtgcaatattccactagaagttatcatttggaacaataacggctacactattgaaagagccatcatgggccctaccaggtcgtataacgacgttatgtcttggaaatggaccaaactatttgaagcattcggagacttcgacggaaagtatactaatagcactctcattcaatgtccctctaaattagcactgaaattggaggagcttaagaattcaaacaaaagaagcgggatagaacttttagaagtcaaattaggcgaattggatttccccgaacagctaaagtgcatggttgaagcagcggcacttaaaagaaataaaaaataggagctctaagaaggagatataccatgaagatcaaagctgttggtgcatattccgctaaacaaccacttgaaccgatggatatcacccggcgtgaaccgggaccgaatgatgtcaaaatcgaaatcgcttactgtggcgtttgccattccgatctccaccaggtccgttccgagtgggcggggacggtttacccctgcgtgccgggtcatgaaattgtggggcgtgtggtagccgttggtgatcaggtagaaaaatatgcgccgggcgatctggtcggtgtcggctgcattgtcgacagttgtaaacattgcgaagagtgtgaagacgggttggaaaactactgtgatcacatgaccggcacctataactcgccgacgccggacgaaccgggccatactctgggcggctactcacaacagatcgtcgttcatgagcgatatgttctgcgtattcgtcacccgcaagagcagctggcggcggtggctcctttgttgtgtgcagggatcaccacgtattcgccgctacgtcactggcaggccgggccgggtaaaaaagtgggcgtggtcggcatcggcggtctgggacatatggggattaagctggcccacgcgatgggggcacatgtggtggcatttaccacttctgaggcaaaacgcgaagcggcaaaagccctgggggccgatgaagttgttaactcacgcaatgccgatgagatggcggctcatctgaagagtttcgatttcattttgaatacagtagctgcgccacataatctcgacgattttaccaccttgctgaagcgtgatggcaccatgacgctggttggtgcgcctgcgacaccgcataaatcgccggaagttttcaacctgatcatgaaacgccgtgcgatagccggttctatgattggcggcattccagaaactcaggagatgctcgatttttgcgccgaacatggcatcgtggctgatatagagatgattcgggccgatcaaattaatgaagcctatgagcgaatgctgcgcggtgatgtgaaatatcgttttgttatcgataatcgcacactaacagactgaggtaccctcgagtctggttaaggtaccctgcagactagtgctattcctgccctttggtcgaaaaaaaaagcccgcactgtcaggtgcgggcttttttctgtgtttcctgc

SEQ ID NO: 106 - DNA, 5215 bp, synthetic construct; identical to SEQ ID NO: 104
  source 1..5215: mol_type = other DNA

SEQ ID NO: 107 - DNA, 4847 bp, synthetic construct
  source 1..4847: mol_type = other DNA
tctagagcttgtcgacgtctcgagccaattattgaaggcctccctaacggggggcctttttttgtttctggtctcccggtctcccgcttaacgatcgttggctgattggatccaattgacagctagctcagtcctaggtaccattggatccaatagctgtcaccggatgtgctttccggtctgatgagtccgtgaggacgaaacagcctctacaaataattttgtttaatactagagaaagaggggaaatactagatggtgtttcaaaaagttgacgcctacgctggcgacccgattcttacgcttatggagcgttttaaagaagaccctcgcagcgacaaagtgaatttaagtatcggtctgtactacaacgaagacggaattattccacaactgcaagccgtggcggaggcggaagcgcgcctgaatgcgcagcctcatggcgcttcgctttatttaccgatggaagggcttaacagctatcgccatgccattgcgccgctgctgtttggtgcggaccatccggtactgaaacaacagcgcgtagcaaccattcaaacccttggcggctccggggcattgaaagtgggcgcggatttcctgaaacgctacttcccggaatcaggcgtctgggtcagcgatcctacctgggaaaaccacgtagcaatattcgccggggctggattcgaagtgagtacttacccctggtatgacgaagcgactaacggcgtgcgctttaatgacctgttggcgacgctgaaaacattacctgcccgcagtattgtgttgctgcatccatgttgccacaacccaacgggtgccgatctcactaatgatcagtgggatgcggtgattgaaattctcaaagcccgcgagcttattccattcctcgatattgcctatcaaggatttggtgccggtatggaagaggatgcctacgctattcgcgccattgccagcgctggattacccgctctggtgagcaattcgttctcgaaaattttctccctttacggcgagcgcgtcggcggactttctgttatgtgtgaagatgccgaagccgctggccgcgtactggggcaattgaaagcaacagttcgccgcaactactccagcccgccgaattttggtgcgcaggtggtggctgcagtgctgaatgacgaggcattgaaagccagctggctggcggaagtagaagagatgcgtactcgcattctggcaatgcgtcaggaattggtgaaggtattaagcacagagatgccagaacgcaatttcgattatctgcttaatcagcgcggcatgttcagttataccggtttaagtgccgctcaggttgaccgactacgtgaagaatttggtgtctatctcatcgccagcggtcgcatgtgtgtcgccgggttaaatacggcaaatgtacaacgtgtggcaaaggcgtttgctgcggtgatgtaaaagctttaagaaggagatataccatgctttttgataacaaaaatcgcggtgctttaaactcactgaacacaccagatattgcttctttatcaatatcatccatgtcggactatcacgtgtttgattttcccggtaaggacctgcagagagaggaagtgatagatttgctagatcagcaagggtttattcccgacgatttgatcgaacaagaagtagattggttttataactcattgggtattgacgatttgttcttctcgagagaatctccccaattaatctcgaatatcatacattctttgtatgcttcaaagctagatttctttgcgaagtccaaattcaacggaattcagccaaggctattcagcattaaaaacaaaattataactaatgataatcatgccatctttatggaatctaatactggtgtcagcataagcgattctcagcaaaaaaactttaaatttgctagtgacgccgtcggaaacgatactttggagcatggtaaggataccatcaaaaaaaataggattgaaatggatgattcttgtccaccttatgaattagattccgaaattgatgaccttttcctggataacaagtctcaaaaaaactgcagattagtttctttttgggctccagaaagcgaattaaagctaacttttgtttatgagagtgtttaccctaatgatgatccagccggcgtagatatttcctctcaggatttgctgaaaggtgatattgaatcgattagtgataagaccatgtacaaagtttcgtcgaacgaaaataaaaaactatacggtctcttacttaagttggttaaagaaagagaaggtcctgtcattaagactactcgctccgtagaaaataaggatgaaattaggttattagtcgcttacaagcgattcaccactaagcgttattactctgctttgaactctttgttccactattacaagttgaaaccttctaagttctatttagagtcgtttaatgttaaggatgatgacatcattatcttttccgtttatttgaacgagaaccagcaattggaagatgttctacttcacgatgtggaggcagcattgaaacaggttgaaagagaagcttcattgctatacgctatcccaaacaattctttccatgaggtttaccagagacgtcaattctcgcccaaagaagctatatatgctcatattggtgctatattcattaaccattttgttaatcgtttaggctctgattatcaaaaccttttatctcaaatcaccattaagcgtaatgatactactcttttggagattgtagaaaacctaaaaagaaagttaagaaatgaaaccttaactcagcaaactattatcaacatcatgtcgaagcattacactataatttccaagttgtataaaaattttgctcaaattcactattatcataatagtactaaagatatggagaagacattatcttttcaaagactggaaaaagtggagccttttaagaatgaccaagagttcgaagcttacttgaataaattcattccaaatgattcacctgatttgttgatcctgaaaacactgaacatcttcaacaagtctattttgaagacaaatttctttattacaagaaaagtagcaatatcattcagattagatccttccctggtgatgacaaaattcgaatatccagagacaccctatggtatattttttgtcgttggtaatactttcaaagggttccatatcaggttcagagatatcgcaaggggcggtattcgtatagtctgttccaggaatcaggatatttatgatttgaattccaagaacgttattgatgagaactatcaattggcctctactcagcaacgtaaaaataaggatattccagagggtggctctaaaggtgtcatcttattgaacccaggattggtagaacatgaccagacatttgtcgccttttcccaatatgtggatgcaatgattgacattctaatcaacgatccattaaaggaaaactatgtcaaccttttaccaaaggaggaaatattattttttggcccagatgaaggaactgctggtttcgtggattgggcaactaaccatgctcgtgtgaggaactgcccatggtggaaatcatttttgactggaaaatccccatctttgggtggtattccccatgacgaatatggtatgacttctctgggtgttcgtgcttatgttaataaaatttacgaaactttaaacttgacaaattctactgtttacaaattccaaactggtggtccggatggtgatttgggatccaatgaaattcttttatcttcgccaaacgaatgttatttggcaattctggacggttcaggtgtcctgtgtgatcctaaaggtttagataaagatgaattatgccgcttggcacatgaaaggaaaatgatttccgatttcgacacttccaaattatcaaacaacggattttttgtttctgtggatgcaatggatatcatgctaccaaatggtacaattgtagctaacggcacaaccttcagaaacacctttcatactcaaattttcaaatttgtggatcatgtcgacatttttgttccatgcggtggtagaccaaactcaattactctaaataatctacattattttgttgacgaaaagactgggaaatgtaaaattccatatattgtggagggtgccaatctatttataacgcaacctgctaaaaatgctttggaggaacatggctgtattctgttcaaagatgcttctgcaaacaaaggtggtgtcacatcttcatcaatggaagtgttggcctcactagcgcttaacgataacgacttcgtgcacaaatttattggagatgttagtggtgagaggtctgcgttgtacaagtcgtacgttgtagaagtgcagtcaagaattcagaaaaatgctgaattagagtttggtcagttatggaatttgaatcaactaaatggaacccacatttcagaaatttcaaaccaattgtccttcactataaacaaattgaacgacgatctagttgcttctcaagagttgtggctcaatgatctaaaattaagaaactacctattgttggataaaataattccaaaaattctgattgatgttgctgggcctcagtccgtattggaaaacattccagagagctatttgaaagttcttctgtcgagttacttatcaagcacttttgtttaccagaacggtatcgatgttaacattggaaaattcttggaatttattggtgggttaaaaagagaagcggaggcaagtgcttgagtaaggtaccctgcagactagtgctattcctgccctttggtcgaaaaaaaaagcccgcactgtcaggtgcgggcttttttctgtgtttcctgc

SEQ ID NO: 108 - DNA, 3326 bp, synthetic construct
  source 1..3326: mol_type = other DNA
ccaattattgaaggcctccctaacggggggcctttttttgtttctggtctcccggtctcccgcttaacgatcgttggctgattggatccaattgacagctagctcagtcctaggtaccattggatccaatagctgtcaccggatgtgctttccggtctgatgagtccgtgaggacgaaacagcctctacaaataattttgtttaatactagagaaagaggggaaatactagatggcacctgttacaattgaaaagttcgtaaatcaagaagaacgacaccttgtttccaaccgatcagcaacaattccgtttggtgaatacatatttaaaagattgttgtccatcgatacgaaatcagttttcggtgttcctggtgacttcaacttatctctattagaatatctctattcacctagtgttgaatcagctggcctaagatgggtcggcacgtgtaatgaactgaacgccgcttatgcggccgacggatattcccgttactctaataagattggctgtttaataaccacgtatggcgttggtgaattaagcgccttgaacggtatagccggttcgttcgctgaaaatgtcaaagttttgcacattgttggtgtggccaagtccatagattcgcgttcaagtaactttagtgatcggaacctacatcatttggtcccacagctacatgattcaaattttaaagggccaaatcataaagtatatcatgatatggtaaaagatagagtcgcttgctcggtagcctacttggaggatattgaaactgcatgtgaccaagtcgataatgttatccgcgatatttacaagtattctaaacctggttatatttttgttcctgcagattttgcggatatgtctgttacatgtgataatttggttaatgttccacgtatatctcaacaagattgtatagtatacccttctgaaaaccaattgtctgacataatcaacaagattactagttggatatattccagtaaaacacctgcgatccttggagacgtactgactgataggtatggtgtgagtaactttttgaacaagcttatctgcaaaactgggatttggaatttttccactgttatgggaaaatctgtaattgatgagtcaaacccaacttatatgggtcaatataatggtaaagaaggtttaaaacaagtctatgaacattttgaactgtgcgacttggtcttgcattttggagtcgacatcaatgaaattaataatgggcattatacttttacttataaaccaaatgctaaaatcattcaatttcatccgaattatattcgccttgtggacactaggcagggcaatgagcaaatgttcaaaggaatcaattttgcccctattttaaaagaactatacaagcgcattgacgtttctaaactttctttgcaatatgattcaaatgtaactcaatatacgaacgaaacaatgcggttagaagatcctaccaatggacaatcaagcattattacacaagttcacttacaaaagacgatgcctaaatttttgaaccctggtgatgttgtcgtttgtgaaacaggctcttttcaattctctgttcgtgatttcgcgtttccttcgcaattaaaatatatatcgcaaggatttttcctttccattggcatggcccttcctgccgccctaggtgttggaattgccatgcaagaccactcaaacgctcacatcaatggtggcaacgtaaaagaggactataagccaagattaattttgtttgaaggtgacggtgcagcacagatgacaatccaagaactgagcaccattctgaagtgcaatattccactagaagttatcatttggaacaataacggctacactattgaaagagccatcatgggccctaccaggtcgtataacgacgttatgtcttggaaatggaccaaactatttgaagcattcggagacttcgacggaaagtatactaatagcactctcattcaatgtccctctaaattagcactgaaattggaggagcttaagaattcaaacaaaagaagcgggatagaacttttagaagtcaaattaggcgaattggatttccccgaacagctaaagtgcatggttgaagcagcggcacttaaaagaaataaaaaataggagctctaagaaggagatataccatgaagatcaaagctgttggtgcatattccgctaaacaaccacttgaaccgatggatatcacccggcgtgaaccgggaccgaatgatgtcaaaatcgaaatcgcttactgtggcgtttgccattccgatctccaccaggtccgttccgagtgggcggggacggtttacccctgcgtgccgggtcatgaaattgtggggcgtgtggtagccgttggtgatcaggtagaaaaatatgcgccgggcgatctggtcggtgtcggctgcattgtcgacagttgtaaacattgcgaagagtgtgaagacgggttggaaaactactgtgatcacatgaccggcacctataactcgccgacgccggacgaaccgggccatactctgggcggctactcacaacagatcgtcgttcatgagcgatatgttctgcgtattcgtcacccgcaagagcagctggcggcggtggctcctttgttgtgtgcagggatcaccacgtattcgccgctacgtcactggcaggccgggccgggtaaaaaagtgggcgtggtcggcatcggcggtctgggacatatggggattaagctggcccacgcgatgggggcacatgtggtggcatttaccacttctgaggcaaaacgcgaagcggcaaaagccctgggggccgatgaagttgttaactcacgcaatgccgatgagatggcggctcatctgaagagtttcgatttcattttgaatacagtagctgcgccacataatctcgacgattttaccaccttgctgaagcgtgatggcaccatgacgctggttggtgcgcctgcgacaccgcataaatcgccggaagttttcaacctgatcatgaaacgccgtgcgatagccggttctatgattggcggcattccagaaactcaggagatgctcgatttttgcgccgaacatggcatcgtggctgatatagagatgattcgggccgatcaaattaatgaagcctatgagcgaatgctgcgcggtgatgtgaaatatcgttttgttatcgataatcgcacactaacagactgagtaaggtaccctgcagactagtgctattcctgccctttggtcgaaaaaaaaagcccgcactgtcaggtgcgggcttttttctgtgtttcctgctactagaagcggccgctgcag

SEQ ID NO: 109 - DNA, 2918 bp, synthetic construct
  source 1..2918: mol_type = other DNA
tctagagcttgtcgacgtctcgagccaattattgaaggcctccctaacggggggcctttttttgtttctggtctcccggtctcccgcttaacgatcgttggctgattggatccaattgacagctagctcagtcctaggtaccattggatccaatagctgtcaccggatgtgctttccggtctgatgagtccgtgaggacgaaacagcctctacaaataattttgtttaatactagagaaagaggggaaatactagatggcgagcctgagcgataagatgaagacctttaccaaggagaccgaagtgcgtggcatggatatgtttgaccagatcaagaatcacgaacaggttctgttttgcaacgacgaggaaaccggcctgaaggcgatcattgcgattcacaacaccaccctgggtccggcgctgggtggctgccgtatgatgccgtatgcgagcgtggatgcggcgctgaacgatgttctgcgtctgagccgtggcatgacctataagtgcgcggcggcggatgtggattttggtggcggtaaagcggttatcattggtgacccgaccaaggataaacacccggagctgttccgtgcgtttggccagttcgtggaaagcctgcaaggtcgtttttacaccggtaccgacatgggtaccagcccggacgatttcgtgcacgcgctgaaggaaaccaactgcatcgtgggcgttgacgaagtttacggcggtagcggtgatagcagcatcccgaccgcgatgggcgtgatttatggtctggaggcgaccaacgaaaccatttggggcagccgtgatctgcacggtaaacgttacgcgatccagggcctgggcaaagtgggctttaaagttgcggagcgtctgctggaggaaggtgctgacctgatcgtgaccgatattagccaccacagcgttgaaaagctgcaactgaaggcgaaagcgctgggcaccgcggtgaaagcggttagcggtgacgagatttatagcgtggacgcggatgttttcatcccgtgcgcgatcggcggtattctgaacgatgaaaccatcgaacgtctgaaggtgaaagcggtggcgggtagcgcgaacaaccagctgctggagcaccgtcacggcatgagcctgcaccaacgtggtatcctgtacgcgccggactatattgtgaacgcgggcggtctgatccaggttgcggatgagctgtatgaaccgaacaaggaacgtgttctgcaaaaaaccggtgcgatttacaacagcctgctgaacatctatacccagagcgagaacgaacacattaccaccgtgcaagcggcggatcgtttttgcgagaaccgtatccaaacccgtaccaagcgtaacagctttttcacccataccaaacgtccgaagtggagcgtgcgtaaataaaagctttaagaaggagatataccatgaaaaacgcgtcaaccgtatcggaagatactgcgtcgaatcaagagccgacgcttcatcgcggattacataaccgtcatattcaactgattgcgctgggtggcgcaattggtactggtctgtttcttggcattggcccggcgattcagatggcgggtccggctgtattgctgggctacggcgtcgccgggatcatcgctttcctgattatgcgccagctcggcgagatggtggtcgaagagccggtatccggttcatttgcccactttgcctataaatactggggaccgtttgcgggcttcctctctggctggaactactgggtaatgttcgtgctggtgggaatggcagagctgaccgctgcgggcatctatatgcagtactggttcccggatgttccaacgtggatttgggctgccgccttctttattatcatcaacgccgttaacctggtgaacgtgcgcttatatggcgaaaccgagttctggtttgcgctgattaaagtgctggcgatcatcggtatgatcggctttggcctgtggctgctgttttctgggcacggcggtgagaaagccagtatcaataacctctggcgctacggcggtttctttgccaccggctggaatggattgattttgtcgctggcggtaattatgttctccttcggcggtctggagctgattgggattactgcggctgaagcgcgcgatccggaaaaaagcatccctaaagcagtgaatcaggtggtgtatcgcatcctgctgttttatatcggttcactggtggttttactggcgctctacccgtgggtggaagtgaaatccaacagtagcccgtttgtgatgattttccataatctcgacagcaacgtggtagcttctgcgctgaacttcgtcattctggtggcatcgctgtcggtgtataacagcggggtttactctaacagccgcatgctgtttggcctttctgtgcagggtaatgcgccaaagtttttgactcgcgtcagccgtcgcggcgtgccgattaactcgctgatgctttccggagcgatcacttcgctggtggtgttaatcaactatctgctgccgcaaaaagcgtttggtctgctgatggcgctggtggtagcaacgctgctgttgaactggattatgatctgcctggcgcatctgcgttttcgtgcagcgatgcgtcgtcaggggcgtgaaacacagtttaaggcgctgctctatccgttcggcaactatctttgcatcgccttcctcggcatgattttgctgctgatgtgcacgatggatgatatgcgcttgtcagcgattctgctgccggtgtggattgtgttcctgtttgtggcgtttaaaacattgcgtaggaaagtgaattaagtaaggtaccctgcagactagtgctattcctgccctttggtcgaaaaaaaaagcccgcactgtcaggtgcgggcttttttctgtgtttcctgc

SEQ ID NO: 110 - DNA, 2913 bp, synthetic construct
  source 1..2913: mol_type = other DNA
cgtctcttctgcggatgactcaaccatatgaatatcctccttagttcctattccgaagttcctattctctagaaagtataggaacttcgaagcagctccagcctacacacgctagggacgtggagtcgattccttacttcttaaaacgatccaaactaaacggcgttggatcaataacaggtttcttgcccatgacaatatcagcggtcacttcacccgctgccgggccttctgtcataccccacactgttgccgtgttaatcactaagcctgggtattctttgacctcagaaatgataggtaattcatcaaatgttggactcacaacggcaccccaacgttcaacaacttctgatttttcaaatactgggaattctgttttcattctttggaaaacagcatctaagtgttgcgtattttgtgttgccgtggcaactcggaattgttcgaatggtgttttttcatctaaattccaagaggtcggcattttaaatgaattaaatagatcttcaccaatagagaattccaacggtaactctccgccacctaataagtgcataaatttaggccctagcaggaagctatctttgactattgaactcgtaaagatacgtggtgcaacggcataagtaccatccgcttgttcgcggaaatgaataccattaggtaaatgcacattaccacgtggtgcaccaggaacccctgagacacgttgttgtgatagatatacattgagcgttgggatatcaatacccatattgcccataaataaacgcgaccagatacccccagcgagtacaacttgagacgttttaatcgcccctttctcactcaccacatcagagattttaccacccgcagtttcaatacctcttactgcacagttggtataaattttcacaccgatttgtttggcataacgagcgagtgcaggtgtgcctgtttcaggatcaacagagcctgaatcttcttcaaatgcagcaacagtccatggcgtttgagcaccgactaagcgatttgatagctcttcacctttaatgatgcgagtatttaatggtgtatcaaaacctgccgcttctttagctgttttgatccacgcttgagctttatctaatgctttttcatctgccagcgcttctacacgaccttgagtacgataactggtatccgcaccaattttctcattcatgccacgccataatattttcccataatggtgtaatgggaagatttctggcgatgtttggtaactaataatttggctgtatgcacggcctgattgctcaccggcaatctgacccttttctaagatagtgacactcataccacgttcagcaaggttaatagcggtcatgatcccttgaataccggcaccaataatcactacatctgcttctttaggaagagccccttgcgtaccttcaacaaatgatgctcttgatttagcttccacaaatttgccgtcacggcgaaccattggaactaaagccgcaccacctgctaaaacgcccgcagcaccaacacctaaaagtagctttctccttgaaatgttcatatgtatatctccttcttaaagttaaacaaaattatttctagaggtatggagaaacagtagagagttgcgaaaaaaagcgtcaggctggatccgctaatcttatggataaaaatgctatggcatagcaaagtgtgacgccgtgcaaataatcaatgtggacttttctgccgtgattatagacacttttgttacgcgtttttgtcatggctttggtcccgctttgttacagaatgcttttaataagcggggttaccggttgggttagcgagaagagccagtaaaagacgcagtgacggcaatgtctgatgcaatatggacaattggtttcttctctgaatggcgggagtatgaaaagtatggctgaagcgcaaaatgatcccctgctgccgggatactcgtttaacgcccatctggtggcgggtttaacgccgattgaggccaacggttatctcgatttttttatcgaccgaccgctgggaatgaaaggttatattctcaatctcaccattcgcggtcagggggtggtgaaaaatcagggacgagaatttgtctgccgaccgggtgatattttgctgttcccgcctggagagattcatcactacggtcgtcatccggaggctcacgaatggtatcaccagtgggtttactttcgtccgcgcgcctactggcatgaatggcttaactggccgtcgatatttgccaataccggtttctttcgcccggatgaagcgcaccagccgcatttcagcgacctgtttgggcaaatcattaatgccggacaaggggaagggcgctattcggaattgctggcgataaatctgcttgagcaattgttactgcggcgcatggaagcgattaacgagtcgctccatccaccgatggataatcgggtacgcgaggcttgtcagtacatcagcgatcacctggcagacagtaattttgatatcgccagcgtcgcacagcatgtctgcctgtcgccgtcgcgtctgtcgcatttgttccgccagcagttagggattagcgtattaagctggcgcgaggaccagcgcatcagtcaggcgaagctgcttttgagcaccacccggatgcctatcgccaccgtcggtcgcaatgtcggttttgacgatcaactctatttctcgcgagtatttaaaaaatgcaccggggcgagtccgagcgagtttagggcaggttgtgaataacgctgatagtgctagtgtagatcgctactagagccaggcatcaaataaaacgaaaggctcagtcgaaagactgggcctttcgttttatctgttgtttgtcggtgaacgctctctactagagtcacactggctcaccttcgggtgggcctttctgcg

SEQ ID NO: 111 - DNA, 735 bp, synthetic construct; identical to SEQ ID NO: 103
  source 1..735: mol_type = other DNA

SEQ ID NO: 112 - DNA, 20 bp, synthetic construct
  source 1..20: mol_type = other DNA
attgtggaaagaccacaccg

SEQ ID NO: 113 - DNA, 20 bp, synthetic construct
  source 1..20: mol_type = other DNA
gccggaagacactatgaagc

SEQ ID NO: 114 - DNA, 20 bp, synthetic construct
  source 1..20: mol_type = other DNA
acgcgcgcctcttccccttc

SEQ ID NO: 115 - DNA, 20 bp, synthetic construct
  source 1..20: mol_type = other DNA
tcatcagagtaagtcggata

SEQ ID NO: 116 - DNA, 20 bp, synthetic construct
  source 1..20: mol_type = other DNA
tgtgtcgtcgttaactcgcc

SEQ ID NO: 117 - DNA, 20 bp, synthetic construct
  source 1..20: mol_type = other DNA
cgatccgtatccaagtgcgg

SEQ ID NO: 118 - DNA, 20 bp, synthetic construct
  source 1..20: mol_type = other DNA
cgtcgttaccccacatatcc

SEQ ID NO: 119 - DNA, 20 bp, synthetic construct
  source 1..20: mol_type = other DNA
cgtatatcgaagatgtgacg

SEQ ID NO: 120 - DNA, 20 bp, synthetic construct
  source 1..20: mol_type = other DNA
cgaagccgccctgtaaacgg

SEQ ID NO: 121 - DNA, 20 bp, synthetic construct
  source 1..20: mol_type = other DNA
gccggaagacactatgaagc

SEQ ID NO: 122 - DNA, 20 bp, synthetic construct
  source 1..20: mol_type = other DNA
accatctttcagttgatcaa

SEQ ID NO: 123 - DNA, 20 bp, synthetic construct
  source 1..20: mol_type = other DNA
ttcttccaccagtccacctt

SEQ ID NO: 124 - DNA, 20 bp, synthetic construct
  source 1..20: mol_type = other DNA
atattactggaacaacataa

SEQ ID NO: 125 - DNA, 20 bp, synthetic construct
  source 1..20: mol_type = other DNA
gtttaccatacactggcccg

SEQ ID NO: 126 - DNA, 20 bp, synthetic construct
  source 1..20: mol_type = other DNA
ggtaaagaagcgttggtcag

SEQ ID NO: 127 - DNA, 20 bp, synthetic construct
  source 1..20: mol_type = other DNA
cgctttttgaaaatacgcaa

SEQ ID NO: 128 - DNA, 20 bp, synthetic construct
  source 1..20: mol_type = other DNA
gagggtgagccataatgaag

SEQ ID NO: 129 - DNA, 20 bp, synthetic construct
  source 1..20: mol_type = other DNA
ttcgaagacatccagcccgg

SEQ ID NO: 130 - DNA, 20 bp, synthetic construct
  source 1..20: mol_type = other DNA
ccgtgacgttatccgcacca

SEQ ID NO: 131 - DNA, 1100 bp, synthetic construct
  source 1..1100: mol_type = other DNA
atggtgaactgccatgacaggtattcgccccagcaacggaactcacaaggcaccataacgtcccctccctgataagactgatactgtggtcgcggttatgccagttggcatcttcacgtaaatagagcaaatagtcccgcgcctggctggcggtttgccaaagccgttgcgactgctgccagtattgccagccatagagcccacttgcgcttagcatgaccagaatcagcatcgcgaccagcgtttcaatcagcgtataaccacgttgtgttttcatgccggcagtatggagcgaggagaaaaaaagacgagggccagtttctatttcttcggcgcatcttccggactatttacgccgttgcaggacgttgcaaaatttcgggaaggtgtctcgaagaatttaacggagggcaaaaaaaaccgacgcacactggcgtcggctctggcaggatgtttcgtaaggttcctcaggaaacgtgttgctgtgggctgcgacgatatgcccagaccatcatgatcacacccgcgacaatcatcgggatggaaagaatttgccccatgctgatgtactgcacccaggcaccagtaaactgcgcgtcgggctggcggaaaaactcaacaatgatgcgaaacgcgccgtaaccaatcaggaacaagcctgagacagctcccattgggcgcggtttacgaatatacaggttgaggataataaacagcaccacaccttccagcagcagctcgtaaagctgtgatgggtggcgcggcagcacaccgtaagtgtcgaaaatggattgccactgcgggttggtttgcagcagcaaaatatcttctgtacgggagccagggaacagcatggcaaacgggaagttcgggtcaacgcggccccacaattcaccgttaataaagttgcccaggcgcccagcaccaagaccaaacggaatgagtggggcctgcaggaattcaaaaaaagcaccgactcggtgccactttttcaagttgataacggactagccttattttaacttgctatttctagctctaaaaccgggccagtgtatggtaaacactagtattatacctaggactgagctagctgtcaa

SEQ ID NO: 132 - DNA, 1404 bp, synthetic construct
  source 1..1404: mol_type = other DNA
aagttcatccagcatagcgccacggatacgctgcactgcgtaagttgtaaatgccgttccttgtagggcgtcatagcgttcgacggcattaagtaacccaatgccgcccgcctgtagcagatcgtcaagttccacgctcgcgggcagtcgaacctgcaggcgcaatgcttcgtgacgcaccagcgggacataacgctgccacagcgagtgtttatccattacaccttcagcggtatagagtgaattcacgataaacagccctgcgttatatgagttatcggcatgattatccgtttctgcagggtttttaatcggacgattagtgggtgaaatgaggggttatttgggggttaccggtaaattgcgggcagaaaaaaccccgccgttggcggggaagcacgttgctggcaaattaccattcatgttgccggatgcggcgtaaacgccttatccggcctacaaaaatgtgcaaattcaataaattgcaattccccttgtaggcctgataagcgcagcgcatcaggcaatttggcgttgccgtcagtctcagttaatcaggttacggcgagattcgttatcctatattgcaagtcgttgattacgttttgggtttccacccgtcggctcaatcgccgtcaaccctgttatcgtctgtcgtaaaacaacctttagaatttttttcacaaacagccattttttgttagtcgacgaaatactcttttctctgccccttattcccgctattaaaaaaaacaattaaacgtaaactttgcgcaattcaggccgataaccccggtattcgttttacgtgtcgaaagataaaaggaaatcgcatggcaagtatttcatcgctgggagtcgggtcaggtctggatttaagttcaatccttgatagcctcaccgccgcgcaaaaagcgacgctaacccctatttcaaatcagcaatcgtcgtttaccgctaaacttagcgcctacggtacgctgaaaagcgcgctgacgactttccagaccgccaatactgcattgtctaaagccgatcttttttccgctaccagcaccaccagcagcaccaccgcgttcagtgccaccaccgcgggtaatgccatcgccgggaaatacaccatcagcgtcacccatctggcgcaggcgcaaaccctgacaacgcgcaccaccagagacgatacgaaaacggcgatcgccaccagcgacagcaaactcaccattcaacaaggcggctatatactagaagcggccgctgcaggaattcaaaaaaagcaccgactcggtgccactttttcaagttgataacggactagccttattttaacttgctatttctagctctaaaacttgatcaactgaaagatggtactagtattatacctaggactgagctagctgtcaa

SEQ ID NO: 133 - DNA, 1458 bp, synthetic construct
  source 1..1458: mol_type = other DNA
aggtcattcttcacattcagggtctgataggtcagatccagtccactgctccgcccaacatccagccaaagcgtggtgctggccgggttttcgcacacgtcctgataatggccgacaaactccagccgcacacggttgaaatcagtaataaacagcgggttaatgggcatttgtgccagcgtttttttacccaactgttctttggtcactggcagcacgcccatcagttcatcattgagataaacctttaactgcgactggacaggcagtaatgatggcgatggcgtgtattcgaggttgagcatcgccttcgtcaccacttcatcgctgcgcataccaaactcaatgctgccgttcgggttaatgccacgtagcaccatgctgcccggcggcggcgcaatttgcgcaaaggtcagcttcacatcacgggaaggaccgttctgcgccacgactggcgcatctgcgccctgcacgcccggcatcacttgccccacctgcggattttgctccgcctgggcggctacagctggctcagcattgatcagtggttgcgttgctggcgtcgcctgcgtcatgaaagaggggaacgcactcatccccagagccactgcacaaatccagaatatttttcttttcatcgcgttatcatcatgatgcactcccgactggcgttttcagcccggaatagtttaacaggcaccagttagccagcgtcagtatttcttcagccgccagcgcatcactgcgaaattcaccgactggttgcttagctgccagacattcagccatcgcttcatcacgatgaatgagcatcggcagcaatcggcgctggctttgcaaccaaagctggtaaatatcgtcctgaacctggctgccaatacggaagtcattaatcaaaatatgtgcaccatccggcagcgcttgctgatgcagtcggatatggcagttggcatccacattgacgattgccagcgagtgatcgcacaaactcagcagctggtgggttatctgcgaggcatcacgcggtaagtcaattaaaatccactggtaacgcccgctggcttttagttgctgtaagccggagcaaatatcgctcagccgggtttgccagtgctgtggattttcttgttcttcaatggataactgaccaaaaggcagcaaatcgagctgcgaggtatagcgtaacccggcgtcacgccagtcctggccatccagcatagctctggcccaaccctgacggtgggtaaaatcaacgttaaatgacaggcgcaacaagttgtccgggcaggtatatactagaagcggccgctgcaggaattcaaaaaaagcaccgactcggtgccactttttcaagttgataacggactagccttattttaacttgctatttctagctctaaaacaaggtggactggtggaagaaactagtattatacctaggactgagctagctgtcaa